European Patent Specification EP 3 856 226 B1, published February 18, 2026. Title: CELLULAR REPROGRAMMING TO REVERSE AGING AND PROMOTE ORGAN AND TISSUE REGENERATION. Applicant: President and Fellows of Harvard College. Application Not Yet Assigned. The sequence listing filed with the application follows.

SEQUENCE LISTING (122 sequences)

SEQ ID NO: 1 - DNA, 1056 bp, Mus musculus
atggctggacacctggcttcagacttcgccttctcacccccaccaggtgggggtgatgggtcagcagggctggagccgggctgggtggatcctcgaacctggctaagcttccaagggcctccaggtgggcctggaatcggaccaggctcagaggtattggggatctccccatgtccgcccgcatacgagttctgcggagggatggcatactgtggacctcaggttggactgggcctagtcccccaagttggcgtggagactttgcagcctgagggccaggcaggagcacgagtggaaagcaactcagagggaacctcctctgagccctgtgccgaccgccccaatgccgtgaagttggagaaggtggaaccaactcccgaggagtcccaggacatgaaagccctgcagaaggagctagaacagtttgccaagctgctgaagcagaagaggatcaccttggggtacacccaggccgacgtggggctcaccctgggcgttctctttggaaaggtgttcagccagaccaccatctgtcgcttcgaggccttgcagctcagccttaagaacatgtgtaagctgcggcccctgctggagaagtgggtggaggaagccgacaacaatgagaaccttcaggagatatgcaaatcggagaccctggtgcaggcccggaagagaaagcgaactagcattgagaaccgtgtgaggtggagtctggagaccatgtttctgaagtgcccgaagccctccctacagcagatcactcacatcgccaatcagcttgggctagagaaggatgtggttcgagtatggttctgtaaccggcgccagaagggcaaaagatcaagtattgagtattcccaacgagaagagtatgaggctacagggacacctttcccagggggggctgtatcctttcctctgcccccaggtccccactttggcaccccaggctatggaagcccccacttcaccacactctactcagtcccttttcctgagggcgaggcctttccctctgttcccgtcactgctctgggctctcccatgcattcaaac

SEQ ID NO: 2 - protein, 352 aa, Mus musculus
MAGHLASDFAFSPPPGGGDGSAGLEPGWVDPRTWLSFQGPPGGPGIGPGSEVLGISPCPPAYEFCGGMAYCGPQVGLGLVPQVGVETLQPEGQAGARVESNSEGTSSEPCADRPNAVKLEKVEPTPEESQDMKALQKELEQFAKLLKQKRITLGYTQADVGLTLGVLFGKVFSQTTICRFEALQLSLKNMCKLRPLLEKWVEEADNNENLQEICKSETLVQARKRKRTSIENRVRWSLETMFLKCPKPSLQQITHIANQLGLEKDVVRVWFCNRRQKGKRSSIEYSQREEYEATGTPFPGGAVSFPLPPGPHFGTPGYGSPHFTTLYSVPFPEGEAFPSVPVTALGSPMHSN

SEQ ID NO: 3 - DNA, 957 bp, Mus musculus
atgtataacatgatggagacggagctgaagccgccgggcccgcagcaagcttcggggggcggcggcggaggaggcaacgccacggcggcggcgaccggcggcaaccagaagaacagcccggaccgcgtcaagaggcccatgaacgccttcatggtatggtcccgggggcagcggcgtaagatggcccaggagaaccccaagatgcacaactcggagatcagcaagcgcctgggcgcggagtggaaacttttgtccgagaccgagaagcggccgttcatcgacgaggccaagcggctgcgcgctctgcacatgaaggagcacccggattataaataccggccgcggcggaaaaccaagacgctcatgaagaaggataagtacacgcttcccggaggcttgctggcccccggcgggaacagcatggcgagcggggttggggtgggcgccggcctgggtgcgggcgtgaaccagcgcatggacagctacgcgcacatgaacggctggagcaacggcagctacagcatgatgcaggagcagctgggctacccgcagcacccgggcctcaacgctcacggcgcggcacagatgcaaccgatgcaccgctacgacgtcagcgccctgcagtacaactccatgaccagctcgcagacctacatgaacggctcgcccacctacagcatgtcctactcgcagcagggcacccccggtatggcgctgggctccatgggctctgtggtcaagtccgaggccagctccagcccccccgtggttacctcttcctcccactccagggcgccctgccaggccggggacctccgggacatgatcagcatgtacctccccggcgccgaggtgccggagcccgctgcgcccagtagactgcacatggcccagcactaccagagcggcccggtgcccggcacggccattaacggcacactgcccctgtcgcacatg

SEQ ID NO: 4 - protein, 319 aa, Mus musculus
MYNMMETELKPPGPQQASGGGGGGGNATAAATGGNQKNSPDRVKRPMNAFMVWSRGQRRKMAQENPKMHNSEISKRLGAEWKLLSETEKRPFIDEAKRLRALHMKEHPDYKYRPRRKTKTLMKKDKYTLPGGLLAPGGNSMASGVGVGAGLGAGVNQRMDSYAHMNGWSNGSYSMMQEQLGYPQHPGLNAHGAAQMQPMHRYDVSALQYNSMTSSQTYMNGSPTYSMSYSQQGTPGMALGSMGSVVKSEASSSPPVVTSSSHSRAPCQAGDLRDMISMYLPGAEVPEPAAPSRLHMAQHYQSGPVPGTAINGTLPLSHM

SEQ ID NO: 5 - DNA, 1446 bp, Mus musculus
atgaggcagccacctggcgagtctgacatggctgtcagcgacgctctgctcccgtccttctccacgttcgcgtccggcccggcgggaagggagaagacactgcgtccagcaggtgccccgactaaccgttggcgtgaggaactctctcacatgaagcgacttcccccacttcccggccgcccctacgacctggcggcgacggtggccacagacctggagagtggcggagctggtgcagcttgcagcagtaacaacccggccctcctagcccggagggagaccgaggagttcaacgacctcctggacctagactttatcctttccaactcgctaacccaccaggaatcggtggccgccaccgtgaccacctcggcgtcagcttcatcctcgtcttccccagcgagcagcggccctgccagcgcgccctccacctgcagcttcagctatccgatccgggccgggggtgacccgggcgtggctgccagcaacacaggtggagggctcctctacagccgagaatctgcgccacctcccacggcccccttcaacctggcggacatcaatgacgtgagcccctcgggcggcttcgtggctgagctcctgcggccggagttggacccagtatacattccgccacagcagcctcagccgccaggtggcgggctgatgggcaagtttgtgctgaaggcgtctctgaccacccctggcagcgagtacagcagcccttcggtcatcagtgttagcaaaggaagcccagacggcagccaccccgtggtagtggcgccctacagcggtggcccgccgcgcatgtgccccaagattaagcaagaggcggtcccgtcctgcacggtcagccggtccctagaggcccatttgagcgctggaccccagctcagcaacggccaccggcccaacacacacgacttccccctggggcggcagctccccaccaggactacccctacactgagtcccgaggaactgctgaacagcagggactgtcaccctggcctgcctcttcccccaggattccatccccatccggggcccaactaccctcctttcctgccagaccagatgcagtcacaagtcccctctctccattatcaagagctcatgccaccgggttcctgcctgccagaggagcccaagccaaagaggggaagaaggtcgtggccccggaaaagaacagccacccacacttgtgactatgcaggctgtggcaaaacctataccaagagttctcatctcaaggcacacctgcgaactcacacaggcgagaaaccttaccactgtgactgggacggctgtgggtggaaattcgcccgctccgatgaactgaccaggcactaccgcaaacacacagggcaccggccctttcagtgccagaagtgcgacagggccttttccaggtcggaccaccttgccttacacatgaagaggcac

SEQ ID NO: 6 - protein, 482 aa, Mus musculus
MRQPPGESDMAVSDALLPSFSTFASGPAGREKTLRPAGAPTNRWREELSHMKRLPPLPGRPYDLAATVATDLESGGAGAACSSNNPALLARRETEEFNDLLDLDFILSNSLTHQESVAATVTTSASASSSSSPASSGPASAPSTCSFSYPIRAGGDPGVAASNTGGGLLYSRESAPPPTAPFNLADINDVSPSGGFVAELLRPELDPVYIPPQQPQPPGGGLMGKFVLKASLTTPGSEYSSPSVISVSKGSPDGSHPVVVAPYSGGPPRMCPKIKQEAVPSCTVSRSLEAHLSAGPQLSNGHRPNTHDFPLGRQLPTRTTPTLSPEELLNSRDCHPGLPLPPGFHPHPGPNYPPFLPDQMQSQVPSLHYQELMPPGSCLPEEPKPKRGRRSWPRKRTATHTCDYAGCGKTYTKSSHLKAHLRTHTGEKPYHCDWDGCGWKFARSDELTRHYRKHTGHRPFQCQKCDRAFSRSDHLALHMKRH

SEQ ID NO: 7 - DNA, 376 bp, Artificial Sequence
  Synthetic Polynucleotide
tttactccctatcagtgatagagaacgtatgaagagtttactccctatcagtgatagagaacgtatgcagactttactccctatcagtgatagagaacgtataaggagtttactccctatcagtgatagagaacgtatgaccagtttactccctatcagtgatagagaacgtatctacagtttactccctatcagtgatagagaacgtatatccagtttactccctatcagtgatagagaacgtataagctttaggcgtgtacggtgggcgcctataaaagcagagctcgtttagtgaaccgtcagatcgcctggagcaattccacaacacttttgtcttataccaactttccgtaccacttcctaccctcgtaaa

SEQ ID NO: 8 - DNA, 169 bp, Artificial Sequence
  Synthetic Polynucleotide
tgcgcgcagcggccgaccatggcccaacttgtttattgcagcttataatggttacaaataaagcaatagcatcacaaatttcacaaataaagcatttttttcactgcattctagttgtggtttgtccaaactcatcaatgtatcttatcatgtctggatctcggtaccg

SEQ ID NO: 9 - protein, 21 aa, Artificial Sequence
  Synthetic Polypeptide
GSGEGRGSLLTCGDVEENPGP

SEQ ID NO: 10 - DNA, 708 bp, Artificial Sequence
  Synthetic Polynucleotide
atgtctaggctggacaagagcaaagtcataaacggagctctggaattactcaatggtgtcggtatcgaaggcctgacgacaaggaaactcgctcaaaagctgggagttgagcagcctaccctgtactggcacgtgaagaacaagcgggccctgctcgatgccctgccaatcgagatgctggacaggcatcatacccacttctgccccctggaaggcgagtcatggcaagactttctgcggaacaacgccaagtcataccgctgtgctctcctctcacatcgcgacggggctaaagtgcatctcggcacccgcccaacagagaaacagtacgaaaccctggaaaatcagctcgcgttcctgtgtcagcaaggcttctccctggagaacgcactgtacgctctgtccgccgtgggccactttacactgggctgcgtattggaggaacaggagcatcaagtagcaaaagaggaaagagagacacctaccaccgattctatgcccccacttctgagacaagcaattgagctgttcgaccggcagggagccgaacctgccttccttttcggcctggaactaatcatatgtggcctggagaaacagctaaagtgcgaaagcggcgggccgaccgacgcccttgacgattttgacttagacatgctcccagccgatgcccttgacgattttgaccttgacatgctccccgggtaa

SEQ ID NO: 11 - protein, 235 aa, Artificial Sequence
  Synthetic Polypeptide
MSRLDKSKVINGALELLNGVGIEGLTTRKLAQKLGVEQPTLYWHVKNKRALLDALPIEMLDRHHTHFCPLEGESWQDFLRNNAKSYRCALLSHRDGAKVHLGTRPTEKQYETLENQLAFLCQQGFSLENALYALSAVGHFTLGCVLEEQEHQVAKEERETPTTDSMPPLLRQAIELFDRQGAEPAFLFGLELIICGLEKQLKCESGGPTDALDDFDLDMLPADALDDFDLDMLPG

SEQ ID NO: 12 - DNA, 747 bp, Artificial Sequence
  Synthetic Polynucleotide
atgtcccgcttggataagagcaaggtaataaatagcgcactcgaactcctcaacggcgtgggcatcgaaggtctgactactcgaaagctcgcccagaaattgggtgtggagcaacctacattgtattggcatgtcaagaacaaaagagccctgctggacgctcttcctattgaaatgcttgacaggcatcacactcattcctgcccccttgaggtcgagagttggcaagattttctccgaaacaatgcaaagtcctaccgctgcgcacttttgtcccatagggatggagcaaaagtgcacctgggaaccaggccaacagagaaacaatacgagactctcgagaaccagttggctttcttgtgccaacaggggttctcacttgaaaatgccctttacgcactgtcagccgttggacattttaccctggggtgcgttcttgaggagcaagaacatcaggttgctaaggaggagcgcgagactccaaccactgattctatgccacctttgctgaaacaggccattgaacttttcgatagacagggtgctgaacctgcctttctcttcgggttggagctgattatttgtggtctcgaaaaacagctgaaatgtgaaagtggtggccctactgacgccctcgatgatttcgacctggatatgctgccagccgatgcacttgatgatttcgatttggatatgcttccagccgacgcactggacgacttcgatttggacatgcttcccggttaa

SEQ ID NO: 13 - protein, 248 aa, Artificial Sequence
  Synthetic Polypeptide
MSRLDKSKVINSALELLNGVGIEGLTTRKLAQKLGVEQPTLYWHVKNKRALLDALPIEMLDRHHTHSCPLEVESWQDFLRNNAKSYRCALLSHRDGAKVHLGTRPTEKQYETLENQLAFLCQQGFSLENALYALSAVGHFTLGCVLEEQEHQVAKEERETPTTDSMPPLLKQAIELFDRQGAEPAFLFGLELIICGLEKQLKCESGGPTDALDDFDLDMLPADALDDFDLDMLPADALDDFDLDMLPG

SEQ ID NO: 14 - DNA, 1050 bp, Artificial Sequence
  Synthetic Polynucleotide
atgcctttgtatcatgctattgcttcccgtatggctttcattttctcctccttgtataaatcctggttgctgtctctttatgaggagttgtggcccgttgtcaggcaacgtggcgtggtgtgcactgtgtttgctgacgcaacccccactggttggggcattgccaccacctgtcagctcctttccgggactttcgctttccccctccctattgccacggcggaactcatcgccgcctgccttgcccgctgctggacaggggctcggctgttgggcactgacaattccgtggtgttgtcggggaaatcatcgtcctttccttggctgctcgcctgtgttgccacctggattctgcgcgggacgtccttctgctacgtcccttcggccctcaatccagcggaccttccttcccgcggcctgctgccggctctgcggcctcttccgcgtcttcgccttcgccctcagacgagtcggatctccctttgggccgcctccccgcatcgataccgtcgacctcgagacctagaaaaacatggagcaatcacaagtagcaatacagcagctaccaatgctgattgtgcctggctagaagcacaagaggaggaggaggtgggttttccagtcacacctcaggtacctttaagaccaatgacttacaaggcagctgtagatcttagccactttttaaaagaaaaggggggactggaagggctaattcactcccaacgaagacaagatatccttgatctgtggatctaccacacacaaggctacttccctgattggcagaactacacaccagggccagggatcagatatccactgacctttggatggtgctacaagctagtaccagttgagcaagagaaggtagaagaagccaatgaaggagagaacacccgcttgttacaccctgtgagcctgcatgggatggatgacccggagagagaagtattagagtggaggtttgacagccgcctagcatttcatcacatggcccgagagctgcatccggactgtactgggtctctctggttagaccagatctga

SEQ ID NO: 15 - protein, 349 aa, Artificial Sequence
  Synthetic Polypeptide
MPLYHAIASRMAFIFSSLYKSWLLSLYEELWPVVRQRGVVCTVFADATPTGWGIATTCQLLSGTFAFPLPIATAELIAACLARCWTGARLLGTDNSVVLSGKSSSFPWLLACVATWILRGTSFCYVPSALNPADLPSRGLLPALRPLPRLRLRPQTSRISLWAASPHRYRRPRDLEKHGAITSSNTAATNADCAWLEAQEEEEVGFPVTPQVPLRPMTYKAAVDLSHFLKEKGGLEGLIHSQRRQDILDLWIYHTQGYFPDWQNYTPGPGIRYPLTFGWCYKLVPVEQEKVEEANEGENTRLLHPVSLHGMDDPEREVLEWRFDSRLAFHHMARELHPDCTGSLWLDQI

SEQ ID NO: 16 - DNA, 7408 bp, Artificial Sequence
  Synthetic Polynucleotide
ttatgcagtgctgccataaccatgagtgataacactgcggccaacttacttctgacaacgatcggaggaccgaaggagctaaccgcttttttgcacaacatgggggatcatgtaactcgccttgatcgttgggaaccggagctgaatgaagccataccaaacgacgagcgtgacaccacgatgcctgtagtaatggtaacaacgttgcgcaaactattaactggcgaactacttactctagcttcccggcaacaattaatagactggatggaggcggataaagttgcaggaccacttctgcgctcggcccttccggctggctggtttattgctgataaatctggagccggtgagcgtgggtctcgcggtatcattgcagcactggggccagatggtaagccctcccgtatcgtagttatctacacgacggggagtcaggcaactatggatgaacgaaatagacagatcgctgagataggtgcctcactgattaagcattggtaactgtcagaccaagtttactcatatatactttagattgatttaaaacttcatttttaatttaaaaggatctaggtgaagatcctttttgataatctcatgaccaaaatcccttaacgtgagttttcgttccactgagcgtcagaccccgtagaaaagatcaaaggatcttcttgagatcctttttttctgcgcgtaatctgctgcttgcaaacaaaaaaaccaccgctaccagcggtggtttgtttgccggatcaagagctaccaactctttttccgaaggtaactggcttcagcagagcgcagataccaaatactgtccttctagtgtagccgtagttaggccaccacttcaagaactctgtagcaccgcctacatacctcgctctgctaatcctgttaccagtggctgctgccagtggcgataagtcgtgtcttaccgggttggactcaagacgatagttaccggataaggcgcagcggtcgggctgaacggggggttcgtgcacacagcccagcttggagcgaacgacctacaccgaactgagatacctacagcgtgagctatgagaaagcgccacgcttcccgaagggagaaaggcggacaggtatccggtaagcggcagggtcggaacaggagagcgcacgagggagcttccagggggaaacgcctggtatctttatagtcctgtcgggtttcgccacctctgacttgagcgtcgatttttgtgatgctcgtcaggggggcggagcctatggaaaaacgccagcaacgcggcctttttacggttcctggccttttgctggccttttgctcacatgttctttcctgcgttatcccctgattctgtggataaccgtattaccgcctttgagtgagctgataccgctcgccgcagccgaacgaccgagcgcagcgagtcagtgagcgaggaagcggaagagcgcccaatacgcaaaccgcctctccccgcgcgttggccgattcattaatgcagctggcacgacaggtttcccgactggaaagcgggcagtgagcgcaacgcaattaatgtgagttagctcactcattaggcaccccaggctttacactttatgcttccggctcgtatgttgtgtggaattgtgagcggataacaatttcacacaggaaacagctatgaccatgattacgccagatttaattaaggccttaattaggctgcgcgctcgctcgctcactgaggccgcccgggcaaagcccgggcgtcgggcgacctttggtcgcccggcctcagtgagcgagcgagcgcgcagagagggagtggccaactccatcactaggggttccttgtagttaatgattaacccgccatgctacttatctacgtagccatgctctaggaagatcggaattctttactccctatcagtgatagagaacgtatgaagagtttactccctatcagtgatagagaacgtatgcagactttactccctatcagtgatagagaacgtataaggagtttactccctatcagtgatagagaacgtatgaccagtttactccctatcagtgatagagaacgtatctacagtttactccctatcagtgatagagaacgtatatccagtttactccctatcagtgatagagaacgtataagctttaggcgtgtacggtgggcgcctataaaagcagagctcgtttagtgaaccgtcagatcgcctggagcaattccacaacacttttgtcttataccaactttccgtaccacttcctaccctcgtaaagcggccgcgccaccatggctggacacctggcttcagacttcgccttctcacccccaccaggtgggggtgatgggtcagcagggctggagccgggctgggtggatcctcgaacctggctaagcttccaagggcctccaggtgggcctggaatcggaccaggctcagaggtattggggatctccccatgtccgcccgcatacgagttctgcggagggatggcatactgtggacctcaggttggactgggcctagtcccccaagttggcgtggagactttgcagcctgagggccaggcaggagcacgagtggaaagcaactcagagggaacctcctctgagccctgtgccgaccgccccaatgccgtgaagttggagaaggtggaaccaactcccgaggagtcccaggacatgaaagccctgcagaaggagctagaacagtttgccaagctgctgaagcagaagaggatcaccttggggtacacccaggccgacgtggggctcaccctgggcgttctctttggaaaggtgttcagccagaccaccatctgtcgcttcgaggccttgcagctcagccttaagaacatgtgtaagctgcggcccctgctggagaagtgggtggaggaagccgacaacaatgagaaccttcaggagatatgcaaatcggagaccctggtgcaggcccggaagagaaagcgaactagcattgagaaccgtgtgaggtggagtctggagaccatgtttctgaagtgcccgaagccctccctacagcagatcactcacatcgccaatcagcttgggctagagaaggatgtggttcgagtatggttctgtaaccggcgccagaagggcaaaagatcaagtattgagtattcccaacgagaagagtatgaggctacagggacacctttcccagggggggctgtatcctttcctctgcccccaggtccccactttggcaccccaggctatggaagcccccacttcaccacactctactcagtcccttttcctgagggcgaggcctttccctctgttcccgtcactgctctgggctctcccatgcattcaaacgctagcggcagcggcgccacgaacttctctctgttaaagcaagcaggagatgttgaagaaaaccccgggcctgcatgcatgtataacatgatggagacggagctgaagccgccgggcccgcagcaagcttcggggggcggcggcggaggaggcaacgccacggcggcggcgaccggcggcaaccagaagaacagcccggaccgcgtcaagaggcccatgaacgccttcatggtatggtcccgggggcagcggcgtaagatggcccaggagaaccccaagatgcacaactcggagatcagcaagcgcctgggcgcggagtggaaacttttgtccgagaccgagaagcggccgttcatcgacgaggccaagcggctgcgcgctctgcacatgaaggagcacccggattataaataccggccgcggcggaaaaccaagacgctcatgaagaaggataagtacacgcttcccggaggcttgctggcccccggcgggaacagcatggcgagcggggttggggtgggcgccggcctgggtgcgggcgtgaaccagcgcatggacagctacgcgcacatgaacggctggagcaacggcagctacagcatgatgcaggagcagctgggctacccgcagcacccgggcctcaacgctcacggcgcggcacagatgcaaccgatgcaccgctacgacgtcagcgccctgcagtacaactccatgaccagctcgcagacctacatgaacggctcgcccacctacagcatgtcctactcgcagcagggcacccccggtatggcgctgggctccatgggctctgtggtcaagtccgaggccagctccagcccccccgtggttacctcttcctcccactccagggcgccctgccaggccggggacctccgggacatgatcagcatgtacctccccggcgccgaggtgccggagcccgctgcgcccagtagactgcacatggcccagcactaccagagcggcccggtgcccggcacggccattaacggcacactgcccctgtcgcacatggcatgcggctccggcgagggcaggggaagtcttctaacatgcggggacgtggaggaaaatcccggcccactcgagatgaggcagccacctggcgagtctgacatggctgtcagcgacgctctgctcccgtccttctccacgttcgcgtccggcccggcgggaagggagaagacactgcgtccagcaggtgccccgactaaccgttggcgtgaggaactctctcacatgaagcgacttcccccacttcccggccgcccctacgacctggcggcgacggtggccacagacctggagagtggcggagctggtgcagcttgcagcagtaacaacccggccctcctagcccggagggagaccgaggagttcaacgacctcctggacctagactttatcctttccaactcgctaacccaccaggaatcggtggccgccaccgtgaccacctcggcgtcagcttcatcctcgtcttccccagcgagcagcggccctgccagcgcgccctccacctgcagcttcagctatccgatccgggccgggggtgacccgggcgtggctgccagcaacacaggtggagggctcctctacagccgagaatctgcgccacctcccacggcccccttcaacctggcggacatcaatgacgtgagcccctcgggcggcttcgtggctgagctcctgcggccggagttggacccagtatacattccgccacagcagcctcagccgccaggtggcgggctgatgggcaagtttgtgctgaaggcgtctctgaccacccctggcagcgagtacagcagcccttcggtcatcagtgttagcaaaggaagcccagacggcagccaccccgtggtagtggcgccctacagcggtggcccgccgcgcatgtgccccaagattaagcaagaggcggtcccgtcctgcacggtcagccggtccctagaggcccatttgagcgctggaccccagctcagcaacggccaccggcccaacacacacgacttccccctggggcggcagctccccaccaggactacccctacactgagtcccgaggaactgctgaacagcagggactgtcaccctggcctgcctcttcccccaggattccatccccatccggggcccaactaccctcctttcctgccagaccagatgcagtcacaagtcccctctctccattatcaagagctcatgccaccgggttcctgcctgccagaggagcccaagccaaagaggggaagaaggtcgtggccccggaaaagaacagccacccacacttgtgactatgcaggctgtggcaaaacctataccaagagttctcatctcaaggcacacctgcgaactcacacaggcgagaaaccttaccactgtgactgggacggctgtgggtggaaattcgcccgctccgatgaactgaccaggcactaccgcaaacacacagggcaccggccctttcagtgccagaagtgcgacagggccttttccaggtcggaccaccttgccttacacatgaagaggcactaaatgactagtgcgcgcagcggccgaccatggcccaacttgtttattgcagcttataatggttacaaataaagcaatagcatcacaaatttcacaaataaagcatttttttcactgcattctagttgtggtttgtccaaactcatcaatgtatcttatcatgtctggatctcggtaccggatccaaattcccgataaggatcttcctagagcatggctacgtagataagtagcatggcgggttaatcattaactacaaggaacccctagtgatggagttggccactccctctctgcgcgctcgctcgctcactgaggccgggcgaccaaaggtcgcccgacgcccgggctttgcccgggcggcctcagtgagcgagcgagcgcgcagccttaattaacctaattcactggccgtcgttttacaacgtcgtgactgggaaaaccctggcgttacccaacttaatcgccttgcagcacatccccctttcgccagctggcgtaatagcgaagaggcccgcaccgatcgcccttcccaacagttgcgcagcctgaatggcgaatgggacgcgccctgtagcggcgcattaagcgcggcgggtgtggtggttacgcgcagcgtgaccgctacacttgccagcgccctagcgcccgctcctttcgctttcttcccttcctttctcgccacgttcgccggctttccccgtcaagctctaaatcgggggctccctttagggttccgatttagtgctttacggcacctcgaccccaaaaaacttgattagggtgatggttcacgtagtgggccatcgccctgatagacggtttttcgccctttgacgttggagtccacgttctttaatagtggactcttgttccaaactggaacaacactcaaccctatctcggtctattcttttgatttataagggattttgccgatttcggcctattggttaaaaaatgagctgatttaacaaaaatttaacgcgaattttaacaaaatattaacgtttataatttcaggtggcatctttcggggaaatgtgcgcggaacccctatttgtttatttttctaaatacattcaaatatgtatccgctcatgagacaataaccctgataaatgcttcaataatattgaaaaaggaagagtatgagtattcaacatttccgtgtcgcccttattcccttttttgcggcattttgccttcctgtttttgctcacccagaaacgctggtgaaagtaaaagatgctgaagatcagttgggtgcacgagtgggttacatcgaactggatctcaatagtggtaagatccttgagagttttcgccccgaagaacgttttccaatgatgagcacttttaaagttctgctatgtggcgcggtattatcccgtattgacgccgggcaagagcaactcggtcgccgcatacactattctcagaatgacttggttgagtactcaccagtcacagaaaagcatcttacggatggcatgacagtaagagaa

SEQ ID NO: 17 - DNA, 5657 bp, Artificial Sequence
  Synthetic Polynucleotide
ttatgcagtgctgccataaccatgagtgataacactgcggccaacttacttctgacaacgatcggaggaccgaaggagctaaccgcttttttgcacaacatgggggatcatgtaactcgccttgatcgttgggaaccggagctgaatgaagccataccaaacgacgagcgtgacaccacgatgcctgtagtaatggtaacaacgttgcgcaaactattaactggcgaactacttactctagcttcccggcaacaattaatagactggatggaggcggataaagttgcaggaccacttctgcgctcggcccttccggctggctggtttattgctgataaatctggagccggtgagcgtgggtctcgcggtatcattgcagcactggggccagatggtaagccctcccgtatcgtagttatctacacgacggggagtcaggcaactatggatgaacgaaatagacagatcgctgagataggtgcctcactgattaagcattggtaactgtcagaccaagtttactcatatatactttagattgatttaaaacttcatttttaatttaaaaggatctaggtgaagatcctttttgataatctcatgaccaaaatcccttaacgtgagttttcgttccactgagcgtcagaccccgtagaaaagatcaaaggatcttcttgagatcctttttttctgcgcgtaatctgctgcttgcaaacaaaaaaaccaccgctaccagcggtggtttgtttgccggatcaagagctaccaactctttttccgaaggtaactggcttcagcagagcgcagataccaaatactgtccttctagtgtagccgtagttaggccaccacttcaagaactctgtagcaccgcctacatacctcgctctgctaatcctgttaccagtggctgctgccagtggcgataagtcgtgtcttaccgggttggactcaagacgatagttaccggataaggcgcagcggtcgggctgaacggggggttcgtgcacacagcccagcttggagcgaacgacctacaccgaactgagatacctacagcgtgagctatgagaaagcgccacgcttcccgaagggagaaaggcggacaggtatccggtaagcggcagggtcggaacaggagagcgcacgagggagcttccagggggaaacgcctggtatctttatagtcctgtcgggtttcgccacctctgacttgagcgtcgatttttgtgatgctcgtcaggggggcggagcctatggaaaaacgccagcaacgcggcctttttacggttcctggccttttgctggccttttgctcacatgttctttcctgcgttatcccctgattctgtggataaccgtattaccgcctttgagtgagctgataccgctcgccgcagccgaacgaccgagcgcagcgagtcagtgagcgaggaagcggaagagcgcccaatacgcaaaccgcctctccccgcgcgttggccgattcattaatgcagctggcacgacaggtttcccgactggaaagcgggcagtgagcgcaacgcaattaatgtgagttagctcactcattaggcaccccaggctttacactttatgcttccggctcgtatgttgtgtggaattgtgagcggataacaatttcacacaggaaacagctatgaccatgattacgccagatttaattaaggccttaattaggctgcgcgctcgctcgctcactgaggccgcccgggcaaagcccgggcgtcgggcgacctttggtcgcccggcctcagtgagcgagcgagcgcgcagagagggagtggccaactccatcactaggggttccttgtagttaatgattaacccgccatgctacttatctacgtagccatgctctaggaagatcggaattcctgatctggcctccgcgccgggttttggcgcctcccgcgggcgcccccctcctcacggcgagcgctgccacgtcagacgaagggcgcagcgagcgtcctgatccttccgcccggacgctcaggacagcggcccgctgctcataagactcggccttagaaccccagtatcagcagaaggacattttaggacgggacttgggtgactctagggcactggttttctttccagagagcggaacaggcgaggaaaagtagtcccttctcggcgattctgcggagggatctccgtggggcggtgaacgccgatgattatataaggacgcgccgggtgtggcacagctagttccgtcgcagccgggatttgggtcgcggttcttgtttgtggatcgctgtgatcgtcacttggtgagtagcgggctgctgggctggccggggctttcgtggccgccgggccgctcggtgggacggaagcgtgtggagagaccgccaagggctgtagtctgggtccgcgagcaaggttgccctgaactgggggttggggggagcgcagcaaaatggcggctgttcccgagtcttgaatggaagacgcttgtgaggcgggctgtgaggtcgttgaaacaaggtggggggcatggtgggcggcaagaacccaaggtcttgaggccttcgctaatgcgggaaagctcttattcgggtgagatgggctggggcaccatctggggaccctgacgtgaagtttgtcactgactggagaactcggtttgtcgtctgttgcgggggcggcagttatgcggtgccgttgggcagtgcacccgtacctttgggagcgcgcgcctcgtcgtgtcgtgacgtcacccgttctgttggcttataatgcagggtggggccacctgccggtaggtgtgcggtaggcttttctccgtcgcaggacgcagggttcgggcctagggtaggctctcctgaatcgacaggcgccggacctctggtgaggggagggataagtgaggcgtcagtttctttggtcggttttatgtacctatcttcttaagtagctgaagctccggttttgaactatgcgctcggggttggcgagtgtgttttgtgaagttttttaggcaccttttgaaatgtaatcatttgggtcaatatgtaattttcagtgttagactagtaaattgtccgctaaattctggccgtttttggcttttttgttagacgaagcggccgcattaaacgccaccatgtcccgcttggataagagcaaggtaataaatagcgcactcgaactcctcaacggcgtgggcatcgaaggtctgactactcgaaagctcgcccagaaattgggtgtggagcaacctacattgtattggcatgtcaagaacaaaagagccctgctggacgctcttcctattgaaatgcttgacaggcatcacactcattcctgcccccttgaggtcgagagttggcaagattttctccgaaacaatgcaaagtcctaccgctgcgcacttttgtcccatagggatggagcaaaagtgcacctgggaaccaggccaacagagaaacaatacgagactctcgagaaccagttggctttcttgtgccaacaggggttctcacttgaaaatgccctttacgcactgtcagccgttggacattttaccctggggtgcgttcttgaggagcaagaacatcaggttgctaaggaggagcgcgagactccaaccactgattctatgccacctttgctgaaacaggccattgaacttttcgatagacagggtgctgaacctgcctttctcttcgggttggagctgattatttgtggtctcgaaaaacagctgaaatgtgaaagtggtggccctactgacgccctcgatgatttcgacctggatatgctgccagccgatgcacttgatgatttcgatttggatatgcttccagccgacgcactggacgacttcgatttggacatgcttcccggttaaactagtctagcaatcaacctctggattacaaaatttgtgaaagattgactggtattcttaactatgttgctccttttacgctatgtggatacgctgctttaatgcctttgtatcatgctattgcttcccgtatggctttcattttctcctccttgtataaatcctggttagttcttgccacggcggaactcatcgccgcctgccttgcccgctgctggacaggggctcggctgttgggcactgacaattccgtggtgtttatttgtgaaatttgtgatgctattgctttatttgtaaccattctagctttatttgtgaaatttgtgatgctattgctttatttgtaaccattataagctgcaataaacaagttaacaacaacaattgcattcattttatgtttcaggttcagggggagatgtgggaggttttttaaagcgggggatccaaattcccgataaggatcttcctagagcatggctacgtagataagtagcatggcgggttaatcattaactacaaggaacccctagtgatggagttggccactccctctctgcgcgctcgctcgctcactgaggccgggcgaccaaaggtcgcccgacgcccgggctttgcccgggcggcctcagtgagcgagcgagcgcgcagccttaattaacctaattcactggccgtcgttttacaacgtcgtgactgggaaaaccctggcgttacccaacttaatcgccttgcagcacatccccctttcgccagctggcgtaatagcgaagaggcccgcaccgatcgcccttcccaacagttgcgcagcctgaatggcgaatgggacgcgccctgtagcggcgcattaagcgcggcgggtgtggtggttacgcgcagcgtgaccgctacacttgccagcgccctagcgcccgctcctttcgctttcttcccttcctttctcgccacgttcgccggctttccccgtcaagctctaaatcgggggctccctttagggttccgatttagtgctttacggcacctcgaccccaaaaaacttgattagggtgatggttcacgtagtgggccatcgccctgatagacggtttttcgccctttgacgttggagtccacgttctttaatagtggactcttgttccaaactggaacaacactcaaccctatctcggtctattcttttgatttataagggattttgccgatttcggcctattggttaaaaaatgagctgatttaacaaaaatttaacgcgaattttaacaaaatattaacgtttataatttcaggtggcatctttcggggaaatgtgcgcggaacccctatttgtttatttttctaaatacattcaaatatgtatccgctcatgagacaataaccctgataaatgcttcaataatattgaaaaaggaagagtatgagtattcaacatttccgtgtcgcccttattcccttttttgcggcattttgccttcctgtttttgctcacccagaaacgctggtgaaagtaaaagatgctgaagatcagttgggtgcacgagtgggttacatcgaactggatctcaatagtggtaagatccttgagagttttcgccccgaagaacgttttccaatgatgagcacttttaaagttctgctatgtggcgcggtattatcccgtattgacgccgggcaagagcaactcggtcgccgcatacactattctcagaatgacttggttgagtactcaccagtcacagaaaagcatcttacggatggcatgacagtaagagaa

SEQ ID NO: 18 - DNA, 1215 bp, Artificial Sequence
  Synthetic Polynucleotide
gatctggcctccgcgccgggttttggcgcctcccgcgggcgcccccctcctcacggcgagcgctgccacgtcagacgaagggcgcagcgagcgtcctgatccttccgcccggacgctcaggacagcggcccgctgctcataagactcggccttagaaccccagtatcagcagaaggacattttaggacgggacttgggtgactctagggcactggttttctttccagagagcggaacaggcgaggaaaagtagtcccttctcggcgattctgcggagggatctccgtggggcggtgaacgccgatgattatataaggacgcgccgggtgtggcacagctagttccgtcgcagccgggatttgggtcgcggttcttgtttgtggatcgctgtgatcgtcacttggtgagtagcgggctgctgggctggccggggctttcgtggccgccgggccgctcggtgggacggaagcgtgtggagagaccgccaagggctgtagtctgggtccgcgagcaaggttgccctgaactgggggttggggggagcgcagcaaaatggcggctgttcccgagtcttgaatggaagacgcttgtgaggcgggctgtgaggtcgttgaaacaaggtggggggcatggtgggcggcaagaacccaaggtcttgaggccttcgctaatgcgggaaagctcttattcgggtgagatgggctggggcaccatctggggaccctgacgtgaagtttgtcactgactggagaactcggtttgtcgtctgttgcgggggcggcagttatgcggtgccgttgggcagtgcacccgtacctttgggagcgcgcgcctcgtcgtgtcgtgacgtcacccgttctgttggcttataatgcagggtggggccacctgccggtaggtgtgcggtaggcttttctccgtcgcaggacgcagggttcgggcctagggtaggctctcctgaatcgacaggcgccggacctctggtgaggggagggataagtgaggcgtcagtttctttggtcggttttatgtacctatcttcttaagtagctgaagctccggttttgaactatgcgctcggggttggcgagtgtgttttgtgaagttttttaggcaccttttgaaatgtaatcatttgggtcaatatgtaattttcagtgttagactagtaaattgtccgctaaattctggccgtttttggcttttttgttagac

SEQ ID NO: 19 - DNA, 19 bp, Artificial Sequence
  Synthetic Polynucleotide
tccctatcagtgatagaga

SEQ ID NO: 20 - DNA, 68 bp, Artificial Sequence
  Synthetic Polynucleotide
gctttaggcgtgtacggtgggcgcctataaaagcagagctcgtttagtgaaccgtcagatcgcctgga

SEQ ID NO: 21 - DNA, 248 bp, Artificial Sequence
  Synthetic Polynucleotide
aatcaacctctggattacaaaatttgtgaaagattgactggtattcttaactatgttgctccttttacgctatgtggatacgctgctttaatgcctttgtatcatgctattgcttcccgtatggctttcattttctcctccttgtataaatcctggttagttcttgccacggcggaactcatcgccgcctgccttgcccgctgctggacaggggctcggctgttgggcactgacaattccgtggtgtt

SEQ ID NO: 22 - DNA, 141 bp, Artificial Sequence
  Synthetic Polynucleotide
ccttaattaggctgcgcgctcgctcgctcactgaggccgcccgggcaaagcccgggcgtcgggcgacctttggtcgcccggcctcagtgagcgagcgagcgcgcagagagggagtggccaactccatcactaggggttcct

SEQ ID NO: 23 - DNA, 438 bp, Artificial Sequence
  Synthetic Polynucleotide
aattcgtacacgcctacctcgacccatcaagtgccacctgacgtctccctatcagtgatagagaagtcgacacgtctcgagctccctatcagtgatagagaaggtacgtctagaacgtctccctatcagtgatagagaagtcgacacgtctcgagctccctatcagtgatagagaaggtacgtctagaacgtctccctatcagtgatagagaagtcgacacgtctcgagctccctatcagtgatagagaaggtacgtctagaacgtctccctatcagtgatagagaagtcgacacgtctcgagctccctatcagtgatagagaaggtaccccctatataagcagagctcgtttagtgaaccgtcagatcgcctggagacgccatccacgctgttttgacctccatagaagacaccgggaccgatccagcctggatcgc

SEQ ID NO: 24 - DNA, 315 bp, Artificial Sequence
  Synthetic Polynucleotide
gagtttactccctatcagtgatagagaacgtatgtcgagtttactccctatcagtgatagagaacgatgtcgagtttactccctatcagtgatagagaacgtatgtcgagtttactccctatcagtgatagagaacgtatgtcgagtttactccctatcagtgatagagaacgtatgtcgagtttatccctatcagtgatagagaacgtatgtcgagtttactccctatcagtgatagagaacgtatgtcgaggtaggcgtgtacggtgggaggcctatataagcagagctcgtttagtgaaccgtcagatcgcc

SEQ ID NO: 25 - DNA, 618 bp, Artificial Sequence
  Synthetic Polynucleotide
atggctagattagataaaagtaaagtgattaacagcgcattagagctgcttaatgaggtcggaatcgaaggtttaacaacccgtaaactcgcccagaagctaggtgtagagcagcctacattgtattggcatgtaaaaaataagcgggctttgctcgacgccttagccattgagatgttagataggcaccatactcacttttgccctttagaaggggaaagctggcaagattttttacgtaataacgctaaaagttttagatgtgctttactaagtcatcgcgatggagcaaaagtacatttaggtacacggcctacagaaaaacagtatgaaactctcgaaaatcaattagcctttttatgccaacaaggtttttcactagagaatgcattatatgcactcagcgctgtggggcattttactttaggttgcgtattggaagatcaagagcatcaagtcgctaaagaagaaagggaaacacctactactgatagtatgccgccattattacgacaagctatcgaattatttgatcaccaaggtgcagagccagccttcttattcggccttgaattgatcatatgcggattagaaaaacaacttaaatgtgaaagtggg

SEQ ID NO: 26 - protein, 206 aa, Artificial Sequence
  Synthetic Polypeptide
MARLDKSKVINSALELLNEVGIEGLTTRKLAQKLGVEQPTLYWHVKNKRALLDALAIEMLDRHHTHFCPLEGESWQDFLRNNAKSFRCALLSHRDGAKVHLGTRPTEKQYETLENQLAFLCQQGFSLENALYALSAVGHFTLGCVLEDQEHQVAKEERETPTTDSMPPLLRQAIELFDHQGAEPAFLFGLELIICGLEKQLKCESG

SEQ ID NO: 27 - DNA, 1008 bp, Artificial Sequence
  Synthetic Polynucleotide
atggctagattagataaaagtaaagtgattaacagcgcattagagctgcttaatgaggtcggaatcgaaggtttaacaacccgtaaactcgcccagaagctaggtgtagagcagcctacattgtattggcatgtaaaaaataagcgggctttgctcgacgccttagccattgagatgttagataggcaccatactcacttttgccctttagaaggggaaagctggcaagattttttacgtaataacgctaaaagttttagatgtgctttactaagtcatcgcgatggagcaaaagtacatttaggtacacggcctacagaaaaacagtatgaaactctcgaaaatcaattagcctttttatgccaacaaggtttttcactagagaatgcattatatgcactcagcgctgtggggcattttactttaggttgcgtattggaagatcaagagcatcaagtcgctaaagaagaaagggaaacacctactactgatagtatgccgccattattacgacaagctatcgaattatttgatcaccaaggtgcagagccagccttcttattcggccttgaattgatcatatgcggattagaaaaacaacttaaatgtgaaagtgggtcgccaaaaaagaagagaaaggtcgacggcggtggtgctttgtctcctcagcactctgctgtcactcaaggaagtatcatcaagaacaaggagggcatggatgctaagtcactaactgcctggtcccggacactggtgaccttcaaggatgtatttgtggacttcaccagggaggagtggaagctgctggacactgctcagcagatcgtgtacagaaatgtgatgctggagaactataagaacctggtttccttgggttatcagcttactaagccagatgtgatcctccggttggagaagggagaagagccctggctggtggagagagaaattcaccaagagacccatcctgattcagagactgcatttgaaatcaaatcatcagtttaa

SEQ ID NO: 28 - protein, 335 aa, Artificial Sequence
  Synthetic Polypeptide
MARLDKSKVINSALELLNEVGIEGLTTRKLAQKLGVEQPTLYWHVKNKRALLDALAIEMLDRHHTHFCPLEGESWQDFLRNNAKSFRCALLSHRDGAKVHLGTRPTEKQYETLENQLAFLCQQGFSLENALYALSAVGHFTLGCVLEDQEHQVAKEERETPTTDSMPPLLRQAIELFDHQGAEPAFLFGLELIICGLEKQLKCESGSPKKKRKVDGGGALSPQHSAVTQGSIIKNKEGMDAKSLTAWSRTLVTFKDVFVDFTREEWKLLDTAQQIVYRNVMLENYKNLVSLGYQLTKPDVILRLEKGEEPWLVEREIHQETHPDSETAFEIKSSV

SEQ ID NO: 29 - DNA, 977 bp, Artificial Sequence
  Synthetic Polynucleotide
accttgcttcctagctgggcctttccttctcctctataaataccagctctggtatttcgccttggcagctgttgctgctagggagacggctggcttgacatgcatctcctgacaaaacacaaacccgtggtgtgagtgggtgtgggcggtgtgagtagggggatgaatcagagagggggcgagggagacaggggcgcaggagtcaggcaaaggcgatgcgggggtgcgactacacgcagttggaaacagtcgtcagaagattctggaaactatcttgctggctataaacttgagggaagcagaaggccaacattcctcccaagggaaactgaggctcagagttaaaacccaggtatcagtgatatgcatgtgccccggccagggtcactctctgactaaccggtacctaccctacaggcctacctagagactcttttgaaaggatggtagagacctgtccgggctttgcccacagtcgttggaaacctcagcattttctaggcaacttgtgcgaataaaacacttcgggggtccttcttgttcattccaataacctaaaacctctcctcggagaaaatagggggcctcaaacaaacgaaattctctagcccgctttccccaggataaggcaggcatccaaatggaaaaaaaggggccggccgggggtctcctgtcagctccttgccctgtgaaacccagcaggcctgcctgtcttctgtcctcttggggctgtccaggggcgcaggcctcttgcgggggagctggcctccccgccccctcgcctgtggccgcccttttcctggcaggacagagggatcctgcagctgtcaggggaggggcgccggggggtgatgtcaggagggctacaaatagtgcagacagctaaggggctccgtcacccatcttcacatccactccagccggctgcccgcccgctgcctcctctgtgcgtccgcccagccagcctcgtccacgcc

SEQ ID NO: 30 - DNA, 5428 bp, Artificial Sequence
  Synthetic Polynucleotide
ttatgcagtgctgccataaccatgagtgataacactgcggccaacttacttctgacaacgatcggaggaccgaaggagctaaccgcttttttgcacaacatgggggatcatgtaactcgccttgatcgttgggaaccggagctgaatgaagccataccaaacgacgagcgtgacaccacgatgcctgtagtaatggtaacaacgttgcgcaaactattaactggcgaactacttactctagcttcccggcaacaattaatagactggatggaggcggataaagttgcaggaccacttctgcgctcggcccttccggctggctggtttattgctgataaatctggagccggtgagcgtgggtctcgcggtatcattgcagcactggggccagatggtaagccctcccgtatcgtagttatctacacgacggggagtcaggcaactatggatgaacgaaatagacagatcgctgagataggtgcctcactgattaagcattggtaactgtcagaccaagtttactcatatatactttagattgatttaaaacttcatttttaatttaaaaggatctaggtgaagatcctttttgataatctcatgaccaaaatcccttaacgtgagttttcgttccactgagcgtcagaccccgtagaaaagatcaaaggatcttcttgagatcctttttttctgcgcgtaatctgctgcttgcaaacaaaaaaaccaccgctaccagcggtggtttgtttgccggatcaagagctaccaactctttttccgaaggtaactggcttcagcagagcgcagataccaaatactgtccttctagtgtagccgtagttaggccaccacttcaagaactctgtagcaccgcctacatacctcgctctgctaatcctgttaccagtggctgctgccagtggcgataagtcgtgtcttaccgggttggactcaagacgatagttaccggataaggcgcagcggtcgggctgaacggggggttcgtgcacacagcccagcttggagcgaacgacctacaccgaactgagatacctacagcgtgagctatgagaaagcgccacgcttcccgaagggagaaaggcggacaggtatccggtaagcggcagggtcggaacaggagagcgcacgagggagcttccagggggaaacgcctggtatctttatagtcctgtcgggtttcgccacctctgacttgagcgtcgatttttgtgatgctcgtcaggggggcggagcctatggaaaaacgccagcaacgcggcctttttacggttcctggccttttgctggccttttgctcacatgttctttcctgcgttatcccctgattctgtggataaccgtattaccgcctttgagtgagctgataccgctcgccgcagccgaacgaccgagcgcagcgagtcagtgagcgaggaagcggaagagcgcccaatacgcaaaccgcctctccccgcgcgttggccgattcattaatgcagctggcacgacaggtttcccgactggaaagcgggcagtgagcgcaacgcaattaatgtgagttagctcactcattaggcaccccaggctttacactttatgcttccggctcgtatgttgtgtggaattgtgagcggataacaatttcacacaggaaacagctatgaccatgattacgccagatttaattaaggccttaattaggctgcgcgctcgctcgctcactgaggccgcccgggcaaagcccgggcgtcgggcgacctttggtcgcccggcctcagtgagcgagcgagcgcgcagagagggagtggccaactccatcactaggggttccttgtagttaatgattaacccgccatgctacttatctacgtagccatgctctaggaagatcggaattcctagatctaccttgcttcctagctgggcctttccttctcctctataaataccagctctggtatttcgccttggcagctgttgctgctagggagacggctggcttgacatgcatctcctgacaaaacacaaacccgtggtgtgagtgggtgtgggcggtgtgagtagggggatgaatcagagagggggcgagggagacaggggcgcaggagtcaggcaaaggcgatgcgggggtgcgactacacgcagttggaaacagtcgtcagaagattctggaaactatcttgctggctataaacttgagggaagcagaaggccaacattcctcccaagggaaactgaggctcagagttaaaacccaggtatcagtgatatgcatgtgccccggccagggtcactctctgactaaccggtacctaccctacaggcctacctagagactcttttgaaaggatggtagagacctgtccgggctttgcccacagtcgttggaaacctcagcattttctaggcaacttgtgcgaataaaacacttcgggggtccttcttgttcattccaataacctaaaacctctcctcggagaaaatagggggcctcaaacaaacgaaattctctagcccgctttccccaggataaggcaggcatccaaatggaaaaaaaggggccggccgggggtctcctgtcagctccttgccctgtgaaacccagcaggcctgcctgtcttctgtcctcttggggctgtccaggggcgcaggcctcttgcgggggagctggcctccccgccccctcgcctgtggccgcccttttcctggcaggacagagggatcctgcagctgtcaggggaggggcgccggggggtgatgtcaggagggctacaaatagtgcagacagctaaggggctccgtcacccatcttcacatccactccagccggctgcccgcccgctgcctcctctgtgcgtccgcccagccagcctcgtccacgccaagcttgcggccgcattaaacgccaccatgtcccgcttggataagagcaaggtaataaatagcgcactcgaactcctcaacggcgtgggcatcgaaggtctgactactcgaaagctcgcccagaaattgggtgtggagcaacctacattgtattggcatgtcaagaacaaaagagccctgctggacgctcttcctattgaaatgcttgacaggcatcacactcattcctgcccccttgaggtcgagagttggcaagattttctccgaaacaatgcaaagtcctaccgctgcgcacttttgtcccatagggatggagcaaaagtgcacctgggaaccaggccaacagagaaacaatacgagactctcgagaaccagttggctttcttgtgccaacaggggttctcacttgaaaatgccctttacgcactgtcagccgttggacattttaccctggggtgcgttcttgaggagcaagaacatcaggttgctaaggaggagcgcgagactccaaccactgattctatgccacctttgctgaaacaggccattgaacttttcgatagacagggtgctgaacctgcctttctcttcgggttggagctgattatttgtggtctcgaaaaacagctgaaatgtgaaagtggtggccctactgacgccctcgatgatttcgacctggatatgctgccagccgatgcacttgatgatttcgatttggatatgcttccagccgacgcactggacgacttcgatttggacatgcttcccggttaaactagtctagcaatcaacctctggattacaaaatttgtgaaagattgactggtattcttaactatgttgctccttttacgctatgtggatacgctgctttaatgcctttgtatcatgctattgcttcccgtatggctttcattttctcctccttgtataaatcctggttagttcttgccacggcggaactcatcgccgcctgccttgcccgctgctggacaggggctcggctgttgggcactgacaattccgtggtgtttatttgtgaaatttgtgatgctattgctttatttgtaaccattctagctttatttgtgaaatttgtgatgctattgctttatttgtaaccattataagctgcaataaacaagttaacaacaacaattgcattcattttatgtttcaggttcagggggagatgtgggaggttttttaaagcgggggatccaaattcccgataaggatcttcctagagcatggctacgtagataagtagcatggcgggttaatcattaactacaaggaacccctagtgatggagttggccactccctctctgcgcgctcgctcgctcactgaggccgggcgaccaaaggtcgcccgacgcccgggctttgcccgggcggcctcagtgagcgagcgagcgcgcagccttaattaacctaattcactggccgtcgttttacaacgtcgtgactgggaaaaccctggcgttacccaacttaatcgccttgcagcacatccccctttcgccagctggcgtaatagcgaagaggcccgcaccgatcgcccttcccaacagttgcgcagcctgaatggcgaatgggacgcgccctgtagcggcgcattaagcgcggcgggtgtggtggttacgcgcagcgtgaccgctacacttgccagcgccctagcgcccgctcctttcgctttcttcccttcctttctcgccacgttcgccggctttccccgtcaagctctaaatcgggggctccctttagggttccgatttagtgctttacggcacctcgaccccaaaaaacttgattagggtgatggttcacgtagtgggccatcgccctgatagacggtttttcgccctttgacgttggagtccacgttctttaatagtggactcttgttccaaactggaacaacactcaaccctatctcggtctattcttttgatttataagggattttgccgatttcggcctattggttaaaaaatgagctgatttaacaaaaatttaacgcgaattttaacaaaatattaacgtttataatttcaggtggcatctttcggggaaatgtgcgcggaacccctatttgtttatttttctaaatacattcaaatatgtatccgctcatgagacaataaccctgataaatgcttcaataatattgaaaaaggaagagtatgagtattcaacatttccgtgtcgcccttattcccttttttgcggcattttgccttcctgtttttgctcacccagaaacgctggtgaaagtaaaagatgctgaagatcagttgggtgcacgagtgggttacatcgaactggatctcaatagtggtaagatccttgagagttttcgccccgaagaacgttttccaatgatgagcacttttaaagttctgctatgtggcgcggtattatcccgtattgacgccgggcaagagcaactcggtcgccgcatacactattctcagaatgacttggttgagtactcaccagtcacagaaaagcatcttacggatggcatgacagtaagagaa

SEQ ID NO: 31 - DNA, 5332 bp, Artificial Sequence
  Synthetic Polynucleotide
aaattgtaaacgttaatattttgttaaaattcgcgttaaatttttgttaaatcagctcattttttaaccaataggccgaaatcggcaaaatcccttataaatcaaaagaatagcccgagatagggttgagtgttgttccagtttggaacaagagtccactattaaagaacgtggactccaacgtcaaagggcgaaaaaccgtctatcagggcgatggcccactacgtgaaccatcacccaaatcaagttttttggggtcgaggtgccgtaaagcactaaatcggaaccctaaagggagcccccgatttagagcttgacggggaaagccggcgaacgtggcgagaaaggaagggaagaaagcgaaaggagcgggcgctagggcgctggcaagtgtagcggtcacgctgcgcgtaaccaccacacccgccgcgcttaatgcgccgctacagggcgcgtactatggttgctttgacgtatgcggtgtgaaataccgcacagatgcgtaaggagaaaataccgcatcaggcgcccctgcaggcagctgcgcgctcgctcgctcactgaggccgcccgggcaaagcccgggcgtcgggcgacctttggtcgcccggcctcagtgagcgagcgagcgcgcagagagggagtggccaactccatcactaggggttcctgcggccgctcggtccgcacgatctcaattcggccattacggccggatccggctcgaggagcttggcccattgcatacgttgtatccatatcataatatgtacatttatattggctcatgtccaacattaccgccatgttgacattgattattgactagttattaatagtaatcaattacggggtcattagttcatagcccatatatggagttccgcgttacataacttacggtaaatggcccgcctggctgaccgcccaacgacccccgcccattgacgtcaataatgacgtatgttcccatagtaacgccaatagggactttccattgacgtcaatgggtggagtatttacgctaaactgcccacttggcagtacatcaagtgtatcatatgccaagtacgccccctattgacgtcaatgacggtaaatggcccgcctggcattatgcccagtacatgaccttatgggactttcctacttggcagtacatctacgtattagtcatcgctattaccatggtgatgcggttttggcagtacatcaatgggcgtggatagcggtttgactcacggggatttccaagtctccaccccattgacgtcaatgggagtttgttttggcaccaaaatcaacgggactttccaaaatgtcgtaacaactccgccccattgacgcaaatgggcggtaggcgtgtacggtgggaggtctatataagcagagctcgtttagtgaaccgtcagatcgcctggagacgccatccacgctgttttgacctccatagaagacaccgggaccgatccagcctccgcggccccgaattcaccatgtctagactggacaagagcaaaatcataaacagcgctctggaattactcaatggagtcggtatcgaaggcctgacgacaaggaaactcgctcaaaagctgggagttgagcagcctaccctgtactggcacgtgaagaacaagcgggccctgctcgatgccctgccaatcgagatgctggacaggcatcatacccacagctgccccctggaaggcgagtcatggcaagactttctgcggaacaacgccaagtcataccgctgtgctctcctctcacatcgcgacggggctaaagtgcatctcggcacccgcccaacagagaaacagtacgaaaccctggaaaatcagctcgcgttcctgtgtcagcaaggcttctccctggagaacgcactgtacgctctgtccgccgtgggccactttacactgggctgcgtattggaggaacaggagcatcaagtagcaaaagaggaaagagagacacctaccaccgattctatgcccccacttctgaagcaagcaattgagctgttcgaccggcagggagccgaacctgccttccttttcggcctggaactaatcatatgtggcctggagaaacagctaaagtgcgaaagcggcgggccgaccgacgcccttgacgattttgacttagacatgctcccagccgatgcccttgacgactttgaccttgatatgctgcctgctgacgctcttgacgattttgaccttgacatgctccccgggtaactaagtaaggatcatcttaattaaatcgataaggatctggccgcctcggcctaatcaacctctggattacaaaatttgtgaaagattgactggtattcttaactatgttgctccttttacgctatgtggatacgctgctttaatgcctttgtatcatgctattgcttcccgtatggctttcattttctcctccttgtataaatcctggttgctgtctctttatgaggagttgtggcccgttgtcaggcaacgtggcgtggtgtgcactgtgtttgctgacgcaacccccactggttggggcattgccaccacctgtcagctcctttccgggactttcgctttccccctccctattgccacggcggaactcatcgccgcctgccttgcccgctgctggacaggggctcggctgttgggcactgacaattccgtggtgttgtcggggaaatcatcgtcctttccttggctgctcgcctgtgttgccacctggattctgcgcgggacgtccttctgctacgtcccttcggccctcaatccagcggaccttccttcccgcggcctgctgccggctctgcggcctcttccgcgtcttcgccttcgccctcagacgagtcggatctccctttgggccgcctccccgccagacatgataagatacattgatgagtttggacaaaccacaactagaatgcagtgaaaaaaatgctttatttgtgaaatttgtgatgctattgctttatttgtaaccattataagctgcaataaacaagttaacaacaacaattgcattcattttatgtttcaggttcagggggagatgtgggaggttttttaaagcaagtaaaacctctacaaatgtggtaactagcgcgtgcggccgcaggaacccctagtgatggagttggccactccctctctgcgcgctcgctcgctcactgaggccgggcgaccaaaggtcgcccgacgcccgggctttgcccgggcggcctcagtgagcgagcgagcgcgcagctgcctgcaggacatgtgagcaaaaggccagcaaaaggccaggaaccgtaaaaaggccgcgttgctggcgtttttccataggctccgcccccctgacgagcatcacaaaaatcgacgctcaagtcagaggtggcgaaacccgacaggactataaagataccaggcgtttccccctggaagctccctcgtgcgctctcctgttccgaccctgccgcttaccggatacctgtccgcctttctcccttcgggaagcgtggcgctttctcatagctcacgctgtaggtatctcagttcggtgtaggtcgttcgctccaagctgggctgtgtgcacgaaccccccgttcagcccgaccgctgcgccttatccggtaactatcgtcttgagtccaacccggtaagacacgacttatcgccactggcagcagccactggtaacaggattagcagagcgaggtatgtaggcggtgctacagagttcttgaagtggtggcctaactacggctacactagaaggacagtatttggtatctgcgctctgctgaagccagttaccttcggaaaaagagttggtagctcttgatccggcaaacaaaccaccgctggtagcggtggtttttttgtttgcaagcagcagattacgcgcagaaaaaaaggatctcaagaagatcctttgatcttttctacggggtctgacgctcagtggaacgaaaactcacgttaagggattttggtcatgagattatcaaaaaggatcttcacctagatccttttaaattaaaaatgaagttttaaatcaatctaaagtatatatgagtaaacttggtctgacagttaccaatgcttaatcagtgaggcacctatctcagcgatctgtctatttcgttcatccatagttgcctgactccccgtcgtgtagataactacgatacgggagggcttaccatctggccccagtgctgcaatgataccgcgagacccacgctcaccggctccagatttatcagcaataaaccagccagccggaagggccgagcgcagaagtggtcctgcaactttatccgcctccatccagtctattaattgttgccgggaagctagagtaagtagttcgccagttaatagtttgcgcaacgttgttgccattgctacaggcatcgtggtgtcacgctcgtcgtttggtatggcttcattcagctccggttcccaacgatcaaggcgagttacatgatcccccatgttgtgcaaaaaagcggttagctccttcggtcctccgatcgttgtcagaagtaagttggccgcagtgttatcactcatggttatggcagcactgcataattctcttactgtcatgccatccgtaagatgcttttctgtgactggtgagtactcaaccaagtcattctgagaatagtgtatgcggcgaccgagttgctcttgcccggcgtcaatacgggataataccgcgccacatagcagaactttaaaagtgctcatcattggaaaacgttcttcggggcgaaaactctcaaggatcttaccgctgttgagatccagttcgatgtaacccactcgtgcacccaactgatcttcagcatcttttactttcaccagcgtttctgggtgagcaaaaacaggaaggcaaaatgccgcaaaaaagggaataagggcgacacggaaatgttgaatactcatactcttcctttttcaatattattgaagcatttatcagggttattgtctcatgagcggatacatatttgaatgtatttagaaaaataaacaaataggggttccgcgcacatttccccgaaaagtgccacctgacgtctaagaaaccattattatcatgacattaacctataaaaataggcgtatcacgaggccctttcgtctcgcgcgtttcggtgatgacggtgaaaacctctgacacatgcagctcccggagacggtcacagcttgtctgtaagcggatgccgggagcagacaagcccgtcagggcgcgtcagcgggtgttggcgggtgtcggggctggcttaactatgcggcatcagagcagattgtactgagagtgcaccata

SEQ ID NO: 32 - DNA, 5392 bp, Artificial Sequence
  Synthetic Polynucleotide
cctgcaggcagctgcgcgctcgctcgctcactgaggccgcccgggcaaagcccgggcgtcgggcgacctttggtcgcccggcctcagtgagcgagcgagcgcgcagagagggagtggccaactccatcactaggggttcctgcggccgcacgcgtggagctagttattaatagtaatcaattacggggtcattagttcatagcccatatatggagttccgcgttacataacttacggtaaatggcccgcctggctgaccgcccaacgacccccgcccattgacgtcaataatgacgtatgttcccatagtaacgtcaatagggactttccattgacgtcaatgggtggagtatttacggtaaactgcccacttggcagtacatcaagtgtatcatatgccaagtacgccccctattgacgtcaatgacggtaaatggcccgcctggcattatgcccagtacatgaccttatgggactttcctacttggcagtacatctacgtattagtcatcgctattaccatggtgatgcggttttggcagtacatcaatgggcgtggatagcggtttgactcacggggatttccaagtctccaccccattgacgtcaatgggagtttgttttgcaccaaaatcaacgggactttccaaaatgtcgtaacaactccgccccattgacgcaaatgggcggtaggcgtgtacggtgggaggtctatataagcagagctcgtttagtgaaccgtcagatcgcctggagacgccatccacgctgttttgacctccatagaagacaccgggaccgatccagcctccgcggattcgaatcccggccgggaacggtgcattggaacgcggattccccgtgccaagagtgacgtaagtaccgcctatagagtctataggcccacaaaaaatgctttcttcttttaatatacttttttgtttatcttatttctaatactttccctaatctctttctttcagggcaataatgatacaatgtatcatgcctctttgcaccattctaaagaataacagtgataatttctgggttaaggcaatagcaatatttctgcatataaatatttctgcatataaattgtaactgatgtaagaggtttcatattgctaatagcagctacaatccagctaccattctgcttttattttatggttgggataaggctggattattctgagtccaagctaggcccttttgctaatcatgttcatacctcttatcttcctcccacagctcctgggcaacgtgctggtctgtgtgctggcccatcactttggcaaagaattgggattcgaacatcgattgaattcatgtctagactggacaagagcaaagtcataaactctgctctggaattactcaatgaagtcggtatcgaaggcctgacgacaaggaaactcgctcaaaagctgggagttgagcagcctaccctgtactggcacgtgaagaacaagcgggccctgctcgatgccctggcaatcgagatgctggacaggcatcatacccacttctgccccctggaaggcgagtcatggcaagactttctgcggaacaacgccaagtcattccgctgtgctctcctctcacatcgcgacggggctaaagtgcatctcggcacccgcccaacagagaaacagtacgaaaccctggaaaatcagctcgcgttcctgtgtcagcaaggcttctccctggagaacgcactgtacgctctgtccgccgtgggccactttacactgggctgcgtattggaggatcaggagcatcaagtagcaaaagaggaaagagagacacctaccaccgattctatgcccccacttctgagacaagcaattgagctgttcgaccatcagggagccgaacctgccttccttttcggcctggaactaatcatatgtggcctggagaaacagctaaagtgcgaaagcggcgggccggccgacgcccttgacgattttgacttagacatgctcccagccgatgcccttgacgactttgaccttgatatgctgcctgctgacgctcttgacgattttgaccttgacatgctccccggatgaggatcctctagagtcgacctgcagaagcttgcctcgagcagcgctgctcgagagatctacgggtggcatccctgtgacccctccccagtgcctctcctggccctggaagttgccactccagtgcccaccagccttgtcctaataaaattaagttgcatcattttgtctgactaggtgtccttctataatattatggggtggaggggggtggtatggagcaaggggcaagttgggaagacaacctgtagggcctgcggggtctattgggaaccaagctggagtgcagtggcacaatcttggctcactgcaatctccgcctcctgggttcaagcgattctcctgcctcagcctcccgagttgttgggattccaggcatgcatgaccaggctcagctaatttttgtttttttggtagagacggggtttcaccatattggccaggctggtctccaactcctaatctcaggtgatctacccaccttggcctcccaaattgctgggattacaggcgtgaaccactgctcccttccctgtccttctgattttgtaggtaaccacgtgcggaccgagcggccgcaggaacccctagtgatggagttggccactccctctctgcgcgctcgctcgctcactgaggccgggcgaccaaaggtcgcccgacgcccgggctttgcccgggcggcctcagtgagcgagcgagcgcgcagctgcctgcaggggcgcctgatgcggtattttctccttacgcatctgtgcggtatttcacaccgcatacgtcaaagcaaccatagtacgcgccctgtagcggcgcattaagcgcggcgggtgtggtggttacgcgcagcgtgaccgctacacttgccagcgccctagcgcccgctcctttcgctttcttcccttcctttctcgccacgttcgccggctttccccgtcaagctctaaatcgggggctccctttagggttccgatttagtgctttacggcacctcgaccccaaaaaacttgatttgggtgatggttcacgtagtgggccatcgccctgatagacggtttttcgccctttgacgttggagtccacgttctttaatagtggactcttgttccaaactggaacaacactcaaccctatctcgggctattcttttgatttataagggattttgccgatttcggcctattggttaaaaaatgagctgatttaacaaaaatttaacgcgaattttaacaaaatattaacgtttacaattttatggtgcactctcagtacaatctgctctgatgccgcatagttaagccagccccgacacccgccaacacccgctgacgcgccctgacgggcttgtctgctcccggcatccgcttacagacaagctgtgaccgtctccgggagctgcatgtgtcagaggttttcaccgtcatcaccgaaacgcgcgagacgaaagggcctcgtgatacgcctatttttataggttaatgtcatgataataatggtttcttagacgtcaggtggcacttttcggggaaatgtgcgcggaacccctatttgtttatttttctaaatacattcaaatatgtatccgctcatgagacaataaccctgataaatgcttcaataatattgaaaaaggaagagtatgagtattcaacatttccgtgtcgcccttattcccttttttgcggcattttgccttcctgtttttgctcacccagaaacgctggtgaaagtaaaagatgctgaagatcagttgggtgcacgagtgggttacatcgaactggatctcaacagcggtaagatccttgagagttttcgccccgaagaacgttttccaatgatgagcacttttaaagttctgctatgtggcgcggtattatcccgtattgacgccgggcaagagcaactcggtcgccgcatacactattctcagaatgacttggttgagtactcaccagtcacagaaaagcatcttacggatggcatgacagtaagagaattatgcagtgctgccataaccatgagtgataacactgcggccaacttacttctgacaacgatcggaggaccgaaggagctaaccgcttttttgcacaacatgggggatcatgtaactcgccttgatcgttgggaaccggagctgaatgaagccataccaaacgacgagcgtgacaccacgatgcctgtagcaatggcaacaacgttgcgcaaactattaactggcgaactacttactctagcttcccggcaacaattaatagactggatggaggcggataaagttgcaggaccacttctgcgctcggcccttccggctggctggtttattgctgataaatctggagccggtgagcgtgggtctcgcggtatcattgcagcactggggccagatggtaagccctcccgtatcgtagttatctacacgacggggagtcaggcaactatggatgaacgaaatagacagatcgctgagataggtgcctcactgattaagcattggtaactgtcagaccaagtttactcatatatactttagattgatttaaaacttcatttttaatttaaaaggatctaggtgaagatcctttttgataatctcatgaccaaaatcccttaacgtgagttttcgttccactgagcgtcagaccccgtagaaaagatcaaaggatcttcttgagatcctttttttctgcgcgtaatctgctgcttgcaaacaaaaaaaccaccgctaccagcggtggtttgtttgccggatcaagagctaccaactctttttccgaaggtaactggcttcagcagagcgcagataccaaatactgtccttctagtgtagccgtagttaggccaccacttcaagaactctgtagcaccgcctacatacctcgctctgctaatcctgttaccagtggctgctgccagtggcgataagtcgtgtcttaccgggttggactcaagacgatagttaccggataaggcgcagcggtcgggctgaacggggggttcgtgcacacagcccagcttggagcgaacgacctacaccgaactgagatacctacagcgtgagctatgagaaagcgccacgcttcccgaagggagaaaggcggacaggtatccggtaagcggcagggtcggaacaggagagcgcacgagggagcttccagggggaaacgcctggtatctttatagtcctgtcgggtttcgccacctctgacttgagcgtcgatttttgtgatgctcgtcaggggggcggagcctatggaaaaacgccagcaacgcggcctttttacggttcctggccttttgctggccttttgctcacatgt

SEQ ID NO: 33 - DNA, 7732 bp, Artificial Sequence
  Synthetic Polynucleotide
ttatgcagtgctgccataaccatgagtgataacactgcggccaacttacttctgacaacgatcggaggaccgaaggagctaaccgcttttttgcacaacatgggggatcatgtaactcgccttgatcgttgggaaccggagctgaatgaagccataccaaacgacgagcgtgacaccacgatgcctgtagtaatggtaacaacgttgcgcaaactattaactggcgaactacttactctagcttcccggcaacaattaatagactggatggaggcggataaagttgcaggaccacttctgcgctcggcccttccggctggctggtttattgctgataaatctggagccggtgagcgtgggtctcgcggtatcattgcagcactggggccagatggtaagccctcccgtatcgtagttatctacacgacggggagtcaggcaactatggatgaacgaaatagacagatcgctgagataggtgcctcactgattaagcattggtaactgtcagaccaagtttactcatatatactttagattgatttaaaacttcatttttaatttaaaaggatctaggtgaagatcctttttgataatctcatgaccaaaatcccttaacgtgagttttcgttccactgagcgtcagaccccgtagaaaagatcaaaggatcttcttgagatcctttttttctgcgcgtaatctgctgcttgcaaacaaaaaaaccaccgctaccagcggtggtttgtttgccggatcaagagctaccaactctttttccgaaggtaactggcttcagcagagcgcagataccaaatactgtccttctagtgtagccgtagttaggccaccacttcaagaactctgtagcaccgcctacatacctcgctctgctaatcctgttaccagtggctgctgccagtggcgataagtcgtgtcttaccgggttggactcaagacgatagttaccggataaggcgcagcggtcgggctgaacggggggttcgtgcacacagcccagcttggagcgaacgacctacaccgaactgagatacctacagcgtgagctatgagaaagcgccacgcttcccgaagggagaaaggcggacaggtatccggtaagcggcagggtcggaacaggagagcgcacgagggagcttccagggggaaacgcctggtatctttatagtcctgtcgggtttcgccacctctgacttgagcgtcgatttttgtgatgctcgtcaggggggcggagcctatggaaaaacgccagcaacgcggcctttttacggttcctggccttttgctggccttttgctcacatgttctttcctgcgttatcccctgattctgtggataaccgtattaccgcctttgagtgagctgataccgctcgccgcagccgaacgaccgagcgcagcgagtcagtgagcgaggaagcggaagagcgcccaatacgcaaaccgcctctccccgcgcgttggccgattcattaatgcagctggcacgacaggtttcccgactggaaagcgggcagtgagcgcaacgcaattaatgtgagttagctcactcattaggcaccccaggctttacactttatgcttccggctcgtatgttgtgtggaattgtgagcggataacaatttcacacaggaaacagctatgaccatgattacgccagatttaattaaggccttaattaggctgcgcgctcgctcgctcactgaggccgcccgggcaaagcccgggcgtcgggcgacctttggtcgcccggcctcagtgagcgagcgagcgcgcagagagggagtggccaactccatcactaggggttccttgtagttaatgattaacccgccatgctacttatctacgtagccatgctctaggaagatcggaattcgtacacgcctacctcgacccatcaagtgccacctgacgtctccctatcagtgatagagaagtcgacacgtctcgagctccctatcagtgatagagaaggtacgtctagaacgtctccctatcagtgatagagaagtcgacacgtctcgagctccctatcagtgatagagaaggtacgtctagaacgtctccctatcagtgatagagaagtcgacacgtctcgagctccctatcagtgatagagaaggtacgtctagaacgtctccctatcagtgatagagaagtcgacacgtctcgagctccctatcagtgatagagaaggtaccccctatataagcagagctcgtttagtgaaccgtcagatcgcctggagacgccatccacgctgttttgacctccatagaagacaccgggaccgatccagcctggatcgcggccgcgccaccatggctggacacctggcttcagacttcgccttctcacccccaccaggtgggggtgatgggtcagcagggctggagccgggctgggtggatcctcgaacctggctaagcttccaagggcctccaggtgggcctggaatcggaccaggctcagaggtattggggatctccccatgtccgcccgcatacgagttctgcggagggatggcatactgtggacctcaggttggactgggcctagtcccccaagttggcgtggagactttgcagcctgagggccaggcaggagcacgagtggaaagcaactcagagggaacctcctctgagccctgtgccgaccgccccaatgccgtgaagttggagaaggtggaaccaactcccgaggagtcccaggacatgaaagccctgcagaaggagctagaacagtttgccaagctgctgaagcagaagaggatcaccttggggtacacccaggccgacgtggggctcaccctgggcgttctctttggaaaggtgttcagccagaccaccatctgtcgcttcgaggccttgcagctcagccttaagaacatgtgtaagctgcggcccctgctggagaagtgggtggaggaagccgacaacaatgagaaccttcaggagatatgcaaatcggagaccctggtgcaggcccggaagagaaagcgaactagcattgagaaccgtgtgaggtggagtctggagaccatgtttctgaagtgcccgaagccctccctacagcagatcactcacatcgccaatcagcttgggctagagaaggatgtggttcgagtatggttctgtaaccggcgccagaagggcaaaagatcaagtattgagtattcccaacgagaagagtatgaggctacagggacacctttcccagggggggctgtatcctttcctctgcccccaggtccccactttggcaccccaggctatggaagcccccacttcaccacactctactcagtcccttttcctgagggcgaggcctttccctctgttcccgtcactgctctgggctctcccatgcattcaaacgctagcggcagcggcgccacgaacttctctctgttaaagcaagcaggagatgttgaagaaaaccccgggcctgcatgcatgtataacatgatggagacggagctgaagccgccgggcccgcagcaagcttcggggggcggcggcggaggaggcaacgccacggcggcggcgaccggcggcaaccagaagaacagcccggaccgcgtcaagaggcccatgaacgccttcatggtatggtcccgggggcagcggcgtaagatggcccaggagaaccccaagatgcacaactcggagatcagcaagcgcctgggcgcggagtggaaacttttgtccgagaccgagaagcggccgttcatcgacgaggccaagcggctgcgcgctctgcacatgaaggagcacccggattataaataccggccgcggcggaaaaccaagacgctcatgaagaaggataagtacacgcttcccggaggcttgctggcccccggcgggaacagcatggcgagcggggttggggtgggcgccggcctgggtgcgggcgtgaaccagcgcatggacagctacgcgcacatgaacggctggagcaacggcagctacagcatgatgcaggagcagctgggctacccgcagcacccgggcctcaacgctcacggcgcggcacagatgcaaccgatgcaccgctacgacgtcagcgccctgcagtacaactccatgaccagctcgcagacctacatgaacggctcgcccacctacagcatgtcctactcgcagcagggcacccccggtatggcgctgggctccatgggctctgtggtcaagtccgaggccagctccagcccccccgtggttacctcttcctcccactccagggcgccctgccaggccggggacctccgggacatgatcagcatgtacctccccggcgccgaggtgccggagcccgctgcgcccagtagactgcacatggcccagcactaccagagcggcccggtgcccggcacggccattaacggcacactgcccctgtcgcacatggcatgcggctccggcgagggcaggggaagtcttctaacatgcggggacgtggaggaaaatcccggcccactcgagatgaggcagccacctggcgagtctgacatggctgtcagcgacgctctgctcccgtccttctccacgttcgcgtccggcccggcgggaagggagaagacactgcgtccagcaggtgccccgactaaccgttggcgtgaggaactctctcacatgaagcgacttcccccacttcccggccgcccctacgacctggcggcgacggtggccacagacctggagagtggcggagctggtgcagcttgcagcagtaacaacccggccctcctagcccggagggagaccgaggagttcaacgacctcctggacctagactttatcctttccaactcgctaacccaccaggaatcggtggccgccaccgtgaccacctcggcgtcagcttcatcctcgtcttccccagcgagcagcggccctgccagcgcgccctccacctgcagcttcagctatccgatccgggccgggggtgacccgggcgtggctgccagcaacacaggtggagggctcctctacagccgagaatctgcgccacctcccacggcccccttcaacctggcggacatcaatgacgtgagcccctcgggcggcttcgtggctgagctcctgcggccggagttggacccagtatacattccgccacagcagcctcagccgccaggtggcgggctgatgggcaagtttgtgctgaaggcgtctctgaccacccctggcagcgagtacagcagcccttcggtcatcagtgttagcaaaggaagcccagacggcagccaccccgtggtagtggcgccctacagcggtggcccgccgcgcatgtgccccaagattaagcaagaggcggtcccgtcctgcacggtcagccggtccctagaggcccatttgagcgctggaccccagctcagcaacggccaccggcccaacacacacgacttccccctggggcggcagctccccaccaggactacccctacactgagtcccgaggaactgctgaacagcagggactgtcaccctggcctgcctcttcccccaggattccatccccatccggggcccaactaccctcctttcctgccagaccagatgcagtcacaagtcccctctctccattatcaagagctcatgccaccgggttcctgcctgccagaggagcccaagccaaagaggggaagaaggtcgtggccccggaaaagaacagccacccacacttgtgactatgcaggctgtggcaaaacctataccaagagttctcatctcaaggcacacctgcgaactcacacaggcgagaaaccttaccactgtgactgggacggctgtgggtggaaattcgcccgctccgatgaactgaccaggcactaccgcaaacacacagggcaccggccctttcagtgccagaagtgcgacagggccttttccaggtcggaccaccttgccttacacatgaagaggcactaaatgactagtctagcaatcaacctctggattacaaaatttgtgaaagattgactggtattcttaactatgttgctccttttacgctatgtggatacgctgctttaatgcctttgtatcatgctattgcttcccgtatggctttcattttctcctccttgtataaatcctggttagttcttgccacggcggaactcatcgccgcctgccttgcccgctgctggacaggggctcggctgttgggcactgacaattccgtggtgtttatttgtgaaatttgtgatgctattgctttatttgtaaccattctagctttatttgtgaaatttgtgatgctattgctttatttgtaaccattataagctgcaataaacaagttaacaacaacaattgcattcattttatgtttcaggttcagggggagatgtgggaggttttttaaagcgggggatccaaattcccgataaggatcttcctagagcatggctacgtagataagtagcatggcgggttaatcattaactacaaggaacccctagtgatggagttggccactccctctctgcgcgctcgctcgctcactgaggccgggcgaccaaaggtcgcccgacgcccgggctttgcccgggcggcctcagtgagcgagcgagcgcgcagccttaattaacctaattcactggccgtcgttttacaacgtcgtgactgggaaaaccctggcgttacccaacttaatcgccttgcagcacatccccctttcgccagctggcgtaatagcgaagaggcccgcaccgatcgcccttcccaacagttgcgcagcctgaatggcgaatgggacgcgccctgtagcggcgcattaagcgcggcgggtgtggtggttacgcgcagcgtgaccgctacacttgccagcgccctagcgcccgctcctttcgctttcttcccttcctttctcgccacgttcgccggctttccccgtcaagctctaaatcgggggctccctttagggttccgatttagtgctttacggcacctcgaccccaaaaaacttgattagggtgatggttcacgtagtgggccatcgccctgatagacggtttttcgccctttgacgttggagtccacgttctttaatagtggactcttgttccaaactggaacaacactcaaccctatctcggtctattcttttgatttataagggattttgccgatttcggcctattggttaaaaaatgagctgatttaacaaaaatttaacgcgaattttaacaaaatattaacgtttataatttcaggtggcatctttcggggaaatgtgcgcggaacccctatttgtttatttttctaaatacattcaaatatgtatccgctcatgagacaataaccctgataaatgcttcaataatattgaaaaaggaagagtatgagtattcaacatttccgtgtcgcccttattcccttttttgcggcattttgccttcctgtttttgctcacccagaaacgctggtgaaagtaaaagatgctgaagatcagttgggtgcacgagtgggttacatcgaactggatctcaatagtggtaagatccttgagagttttcgccccgaagaacgttttccaatgatgagcacttttaaagttctgctatgtggcgcggtattatcccgtattgacgccgggcaagagcaactcggtcgccgcatacactattctcagaatgacttggttgagtactcaccagtcacagaaaagcatcttacggatggcatgacagtaagagaa

SEQ ID NO: 34 - DNA, 186 bp, Artificial Sequence
  Synthetic Polynucleotide
gaggccagcggttccggacgggctgacgcattggacgattttgatctggatatgctgggaagtgacgccctcgatgattttgaccttgacatgcttggttcggatgcccttgatgactttgacctcgacatgctcggcagtgacgcccttgatgatttcgacctggacatgctgattaactctaga

SEQ ID NO: 35 - DNA, 783 bp, Artificial Sequence
  Synthetic Polynucleotide
agccagtacctgcccgacaccgacgaccggcaccggatcgaggaaaagcggaagcggacctacgagacattcaagagcatcatgaagaagtcccccttcagcggccccaccgaccctagacctccacctagaagaatcgccgtgcccagcagatccagcgccagcgtgccaaaacctgccccccagccttaccccttcaccagcagcctgagcaccatcaactacgacgagttccctaccatggtgttccccagcggccagatctctcaggcctctgctctggctccagcccctcctcaggtgctgcctcaggctcctgctcctgcaccagctccagccatggtgtctgcactggctcaggcaccagcacccgtgcctgtgctggctcctggacctccacaggctgtggctccaccagcccctaaacctacacaggccggcgagggcacactgtctgaagctctgctgcagctgcagttcgacgacgaggatctgggagccctgctgggaaacagcaccgatcctgccgtgttcaccgacctggccagcgtggacaacagcgagttccagcagctgctgaaccagggcatccctgtggcccctcacaccaccgagcccatgctgatggaataccccgaggccatcacccggctcgtgacaggcgctcagaggcctcctgatccagctcctgcccctctgggagcaccaggcctgcctaatggactgctgtctggcgacgaggacttcagctctatcgccgatatggatttctcagccttgctg

SEQ ID NO: 36 - DNA, 570 bp, Artificial Sequence
  Synthetic Polynucleotide
cgggattccagggaagggatgtttttgccgaagcctgaggccggctccgctattagtgacgtgtttgagggccgcgaggtgtgccagccaaaacgaatccggccatttcatcctccaggaagtccatgggccaaccgcccactccccgccagcctcgcaccaacaccaaccggtccagtacatgagccagtcgggtcactgaccccggcaccagtccctcagccactggatccagcgcccgcagtgactcccgaggccagtcacctgttggaggatcccgatgaagagacgagccaggctgtcaaagcccttcgggagatggccgatactgtgattccccagaaggaagaggctgcaatctgtggccaaatggacctttcccatccgcccccaaggggccatctggatgagctgacaaccacacttgagtccatgaccgaggatctgaacctggactcacccctgaccccggaattgaacgagattctggataccttcctgaacgacgagtgcctcttgcatgccatgcatatcagcacaggactgtccatcttcgacacatctctgttt

SEQ ID NO: 37 - DNA, 1416 bp, Artificial Sequence
  Synthetic Polynucleotide
gcttcaaactttactcagttcgtgctcgtggacaatggtgggacaggggatgtgacagtggctccttctaatttcgctaatggggtggcagagtggatcagctccaactcacggagccaggcctacaaggtgacatgcagcgtcaggcagtctagtgcccagaagagaaagtataccatcaaggtggaggtccccaaagtggctacccagacagtgggcggagtcgaactgcctgtcgccgcttggaggtcctacctgaacatggagctcactatcccaattttcgctaccaattctgactgtgaactcatcgtgaaggcaatgcaggggctcctcaaagacggtaatcctatcccttccgccatcgccgctaactcaggtatctacagcgctggaggaggtggaagcggaggaggaggaagcggaggaggaggtagcggacctaagaaaaagaggaaggtggcggccgctggatccccttcagggcagatcagcaaccaggccctggctctggcccctagctccgctccagtgctggcccagactatggtgccctctagtgctatggtgcctctggcccagccacctgctccagcccctgtgctgaccccaggaccaccccagtcactgagcgctccagtgcccaagtctacacaggccggcgaggggactctgagtgaagctctgctgcacctgcagttcgacgctgatgaggacctgggagctctgctggggaacagcaccgatcccggagtgttcacagatctggcctccgtggacaactctgagtttcagcagctgctgaatcagggcgtgtccatgtctcatagtacagccgaaccaatgctgatggagtaccccgaagccattacccggctggtgaccggcagccagcggccccccgaccccgctccaactcccctgggaaccagcggcctgcctaatgggctgtccggagatgaagacttctcaagcatcgctgatatggactttagtgccctgctgtcacagatttcctctagtgggcagggaggaggtggaagcggcttcagcgtggacaccagtgccctgctggacctgttcagcccctcggtgaccgtgcccgacatgagcctgcctgaccttgacagcagcctggccagtatccaagagctcctgtctccccaggagccccccaggcctcccgaggcagagaacagcagcccggattcagggaagcagctggtgcactacacagcgcagccgctgttcctgctggaccccggctccgtggacaccgggagcaacgacctgccggtgctgtttgagctgggagagggctcctacttctccgaaggggacggcttcgccgaggaccccaccatctccctgctgacaggctcggagcctcccaaagccaaggaccccactgtctcc

SEQ ID NO: 38 - DNA, 3594 bp, Artificial Sequence
  Synthetic Polynucleotide
atggcgggacacctggcttcggatttcgccttctcgccccctccaggtggtggaggtgatgggccaggggggccggagccgggctgggttgatcctcggacctggctaagcttccaaggccctcctggagggccaggaatcgggccgggggttgggccaggctctgaggtgtgggggattcccccatgccccccgccgtatgagttctgtggggggatggcgtactgtgggccccaggttggagtggggctagtgccccaaggcggcttggagacctctcagcctgagggcgaagcaggagtcggggtggagagcaactccgatggggcctccccggagccctgcaccgtcacccctggtgccgtgaagctggagaaggagaagctggagcaaaacccggaggagtcccaggacatcaaagctctgcagaaagaactcgagcaatttgccaagctcctgaagcagaagaggatcaccctgggatatacacaggccgatgtggggctcaccctgggggttctatttgggaaggtattcagccaaacgaccatctgccgctttgaggctctgcagcttagcttcaagaacatgtgtaagctgcggcccttgctgcagaagtgggtggaggaagctgacaacaatgaaaatcttcaggagatatgcaaagcagaaaccctcgtgcaggcccgaaagagaaagcgaaccagtatcgagaaccgagtgagaggcaacctggagaatttgttcctgcagtgcccgaaacccacactgcagcagatcagccacatcgcccagcagcttgggctcgagaaggatgtggtccgagtgtggttctgtaaccggcgccagaagggcaagcgatcaagcagcgactatgcacaacgagaggattttgaggctgctgggtctcctttctcagggggaccagtgtcctttcctctggccccagggccccattttggtaccccaggctatgggagccctcacttcactgcactgtactcctcggtccctttccctgagggggaagcctttccccctgtctctgtcaccactctgggctctcccatgcattcaaacgctagcggcagcggcgccacgaacttctctctgttaaagcaagcaggagatgttgaagaaaaccccgggcctgcatgcatgtacaacatgatggagacggagctgaagccgccgggcccgcagcaaacttcggggggcggcggcggcaactccaccgcggcggcggccggcggcaaccagaaaaacagcccggaccgcgtcaagcggcccatgaatgccttcatggtgtggtcccgcgggcagcggcgcaagatggcccaggagaaccccaagatgcacaactcggagatcagcaagcgcctgggcgccgagtggaaacttttgtcggagacggagaagcggccgttcatcgacgaggctaagcggctgcgagcgctgcacatgaaggagcacccggattataaataccggccccggcggaaaaccaagacgctcatgaagaaggataagtacacgctgcccggcgggctgctggcccccggcggcaatagcatggcgagcggggtcggggtgggcgccggcctgggcgcgggcgtgaaccagcgcatggacagttacgcgcacatgaacggctggagcaacggcagctacagcatgatgcaggaccagctgggctacccgcagcacccgggcctcaatgcgcacggcgcagcgcagatgcagcccatgcaccgctacgacgtgagcgccctgcagtacaactccatgaccagctcgcagacctacatgaacggctcgcccacctacagcatgtcctactcgcagcagggcacccctggcatggctcttggctccatgggttcggtggtcaagtccgaggccagctccagcccccctgtggttacctcttcctcccactccagggcgccctgccaggccggggacctccgggacatgatcagcatgtatctccccggcgccgaggtgccggaacccgccgcccccagcagacttcacatgtcccagcactaccagagcggcccggtgcccggcacggccattaacggcacactgcccctctcacacatggcatgcggctccggcgagggcaggggaagtcttctaacatgcggggacgtggaggaaaatcccggcccactcgagatggctgtcagcgacgcgctgctcccatctttctccacgttcgcgtctggcccggcgggaagggagaagacactgcgtcaagcaggtgccccgaataaccgctggcgggaggagctctcccacatgaagcgacttcccccagtgcttcccggccgcccctatgacctggcggcggcgaccgtggccacagacctggagagcggcggagccggtgcggcttgcggcggtagcaacctggcgcccctacctcggagagagaccgaggagttcaacgatctcctggacctggactttattctctccaattcgctgacccatcctccggagtcagtggccgccaccgtgtcctcgtcagcgtcagcctcctcttcgtcgtcgccgtcgagcagcggccctgccagcgcgccctccacctgcagcttcacctatccgatccgggccgggaacgacccgggcgtggcgccgggcggcacgggcggaggcctcctctatggcagggagtccgctccccctccgacggctcccttcaacctggcggacatcaacgacgtgagcccctcgggcggcttcgtggccgagctcctgcggccagaattggacccggtgtacattccgccgcagcagccgcagccgccaggtggcgggctgatgggcaagttcgtgctgaaggcgtcgctgagcgcccctggcagcgagtacggcagcccgtcggtcatcagcgtcagcaaaggcagccctgacggcagccacccggtggtggtggcgccctacaacggcgggccgccgcgcacgtgccccaagatcaagcaggaggcggtctcttcgtgcacccacttgggcgctggaccccctctcagcaatggccaccggccggctgcacacgacttccccctggggcggcagctccccagcaggactaccccgaccctgggtcttgaggaagtgctgagcagcagggactgtcaccctgccctgccgcttcctcccggcttccatccccacccggggcccaattacccatccttcctgcccgatcagatgcagccgcaagtcccgccgctccattaccaagagctcatgccacccggttcctgcatgccagaggagcccaagccaaagaggggaagacgatcgtggccccggaaaaggaccgccacccacacttgtgattacgcgggctgcggcaaaacctacacaaagagttcccatctcaaggcacacctgcgaacccacacaggtgagaaaccttaccactgtgactgggacggctgtggatggaaattcgcccgctcagatgaactgaccaggcactaccgtaaacacacggggcaccgcccgttccagtgccaaaaatgcgaccgagcattttccaggtcggaccacctcgccttacacatgaagaggcatttt

SEQ ID NO: 39 - protein, 1198 aa, Artificial Sequence
  Synthetic Polypeptide
MAGHLASDFAFSPPPGGGGDGPGGPEPGWVDPRTWLSFQGPPGGPGIGPGVGPGSEVWGIPPCPPPYEFCGGMAYCGPQVGVGLVPQGGLETSQPEGEAGVGVESNSDGASPEPCTVTPGAVKLEKEKLEQNPEESQDIKALQKELEQFAKLLKQKRITLGYTQADVGLTLGVLFGKVFSQTTICRFEALQLSFKNMCKLRPLLQKWVEEADNNENLQEICKAETLVQARKRKRTSIENRVRGNLENLFLQCPKPTLQQISHIAQQLGLEKDVVRVWFCNRRQKGKRSSSDYAQREDFEAAGSPFSGGPVSFPLAPGPHFGTPGYGSPHFTALYSSVPFPEGEAFPPVSVTTLGSPMHSNASGSGATNFSLLKQAGDVEENPGPACMYNMMETELKPPGPQQTSGGGGGNSTAAAAGGNQKNSPDRVKRPMNAFMVWSRGQRRKMAQENPKMHNSEISKRLGAEWKLLSETEKRPFIDEAKRLRALHMKEHPDYKYRPRRKTKTLMKKDKYTLPGGLLAPGGNSMASGVGVGAGLGAGVNQRMDSYAHMNGWSNGSYSMMQDQLGYPQHPGLNAHGAAQMQPMHRYDVSALQYNSMTSSQTYMNGSPTYSMSYSQQGTPGMALGSMGSVVKSEASSSPPVVTSSSHSRAPCQAGDLRDMISMYLPGAEVPEPAAPSRLHMSQHYQSGPVPGTAINGTLPLSHMACGSGEGRGSLLTCGDVEENPGPLEMAVSDALLPSFSTFASGPAGREKTLRQAGAPNNRWREELSHMKRLPPVLPGRPYDLAAATVATDLESGGAGAACGGSNLAPLPRRETEEFNDLLDLDFILSNSLTHPPESVAATVSSSASASSSSSPSSSGPASAPSTCSFTYPIRAGNDPGVAPGGTGGGLLYGRESAPPPTAPFNLADINDVSPSGGFVAELLRPELDPVYIPPQQPQPPGGGLMGKFVLKASLSAPGSEYGSPSVISVSKGSPDGSHPVVVAPYNGGPPRTCPKIKQEAVSSCTHLGAGPPLSNGHRPAAHDFPLGRQLPSRTTPTLGLEEVLSSRDCHPALPLPPGFHPHPGPNYPSFLPDQMQPQVPPLHYQELMPPGSCMPEEPKPKRGRRSWPRKRTATHTCDYAGCGKTYTKSSHLKAHLRTHTGEKPYHCDWDGCGWKFARSDELTRHYRKHTGHRPFQCQKCDRAFSRSDHLALHMKRHF

SEQ ID NO: 40 - DNA, 1080 bp, Homo sapiens
atggcgggacacctggcttcggatttcgccttctcgccccctccaggtggtggaggtgatgggccaggggggccggagccgggctgggttgatcctcggacctggctaagcttccaaggccctcctggagggccaggaatcgggccgggggttgggccaggctctgaggtgtgggggattcccccatgccccccgccgtatgagttctgtggggggatggcgtactgtgggccccaggttggagtggggctagtgccccaaggcggcttggagacctctcagcctgagggcgaagcaggagtcggggtggagagcaactccgatggggcctccccggagccctgcaccgtcacccctggtgccgtgaagctggagaaggagaagctggagcaaaacccggaggagtcccaggacatcaaagctctgcagaaagaactcgagcaatttgccaagctcctgaagcagaagaggatcaccctgggatatacacaggccgatgtggggctcaccctgggggttctatttgggaaggtattcagccaaacgaccatctgccgctttgaggctctgcagcttagcttcaagaacatgtgtaagctgcggcccttgctgcagaagtgggtggaggaagctgacaacaatgaaaatcttcaggagatatgcaaagcagaaaccctcgtgcaggcccgaaagagaaagcgaaccagtatcgagaaccgagtgagaggcaacctggagaatttgttcctgcagtgcccgaaacccacactgcagcagatcagccacatcgcccagcagcttgggctcgagaaggatgtggtccgagtgtggttctgtaaccggcgccagaagggcaagcgatcaagcagcgactatgcacaacgagaggattttgaggctgctgggtctcctttctcagggggaccagtgtcctttcctctggccccagggccccattttggtaccccaggctatgggagccctcacttcactgcactgtactcctcggtccctttccctgagggggaagcctttccccctgtctctgtcaccactctgggctctcccatgcattcaaac

SEQ ID NO: 41 - protein, 360 aa, Homo sapiens
MAGHLASDFAFSPPPGGGGDGPGGPEPGWVDPRTWLSFQGPPGGPGIGPGVGPGSEVWGIPPCPPPYEFCGGMAYCGPQVGVGLVPQGGLETSQPEGEAGVGVESNSDGASPEPCTVTPGAVKLEKEKLEQNPEESQDIKALQKELEQFAKLLKQKRITLGYTQADVGLTLGVLFGKVFSQTTICRFEALQLSFKNMCKLRPLLQKWVEEADNNENLQEICKAETLVQARKRKRTSIENRVRGNLENLFLQCPKPTLQQISHIAQQLGLEKDVVRVWFCNRRQKGKRSSSDYAQREDFEAAGSPFSGGPVSFPLAPGPHFGTPGYGSPHFTALYSSVPFPEGEAFPPVSVTTLGSPMHSN

SEQ ID NO: 42 - DNA, 951 bp, Homo sapiens
atgtacaacatgatggagacggagctgaagccgccgggcccgcagcaaacttcggggggcggcggcggcaactccaccgcggcggcggccggcggcaaccagaaaaacagcccggaccgcgtcaagcggcccatgaatgccttcatggtgtggtcccgcgggcagcggcgcaagatggcccaggagaaccccaagatgcacaactcggagatcagcaagcgcctgggcgccgagtggaaacttttgtcggagacggagaagcggccgttcatcgacgaggctaagcggctgcgagcgctgcacatgaaggagcacccggattataaataccggccccggcggaaaaccaagacgctcatgaagaaggataagtacacgctgcccggcgggctgctggcccccggcggcaatagcatggcgagcggggtcggggtgggcgccggcctgggcgcgggcgtgaaccagcgcatggacagttacgcgcacatgaacggctggagcaacggcagctacagcatgatgcaggaccagctgggctacccgcagcacccgggcctcaatgcgcacggcgcagcgcagatgcagcccatgcaccgctacgacgtgagcgccctgcagtacaactccatgaccagctcgcagacctacatgaacggctcgcccacctacagcatgtcctactcgcagcagggcacccctggcatggctcttggctccatgggttcggtggtcaagtccgaggccagctccagcccccctgtggttacctcttcctcccactccagggcgccctgccaggccggggacctccgggacatgatcagcatgtatctccccggcgccgaggtgccggaacccgccgcccccagcagacttcacatgtcccagcactaccagagcggcccggtgcccggcacggccattaacggcacactgcccctctcacacatg

SEQ ID NO: 43 - protein, 317 aa, Homo sapiens
MYNMMETELKPPGPQQTSGGGGGNSTAAAAGGNQKNSPDRVKRPMNAFMVWSRGQRRKMAQENPKMHNSEISKRLGAEWKLLSETEKRPFIDEAKRLRALHMKEHPDYKYRPRRKTKTLMKKDKYTLPGGLLAPGGNSMASGVGVGAGLGAGVNQRMDSYAHMNGWSNGSYSMMQDQLGYPQHPGLNAHGAAQMQPMHRYDVSALQYNSMTSSQTYMNGSPTYSMSYSQQGTPGMALGSMGSVVKSEASSSPPVVTSSSHSRAPCQAGDLRDMISMYLPGAEVPEPAAPSRLHMSQHYQSGPVPGTAINGTLPLSHM

SEQ ID NO: 44 - DNA, 1410 bp, Homo sapiens
atggctgtcagcgacgcgctgctcccatctttctccacgttcgcgtctggcccggcgggaagggagaagacactgcgtcaagcaggtgccccgaataaccgctggcgggaggagctctcccacatgaagcgacttcccccagtgcttcccggccgcccctatgacctggcggcggcgaccgtggccacagacctggagagcggcggagccggtgcggcttgcggcggtagcaacctggcgcccctacctcggagagagaccgaggagttcaacgatctcctggacctggactttattctctccaattcgctgacccatcctccggagtcagtggccgccaccgtgtcctcgtcagcgtcagcctcctcttcgtcgtcgccgtcgagcagcggccctgccagcgcgccctccacctgcagcttcacctatccgatccgggccgggaacgacccgggcgtggcgccgggcggcacgggcggaggcctcctctatggcagggagtccgctccccctccgacggctcccttcaacctggcggacatcaacgacgtgagcccctcgggcggcttcgtggccgagctcctgcggccagaattggacccggtgtacattccgccgcagcagccgcagccgccaggtggcgggctgatgggcaagttcgtgctgaaggcgtcgctgagcgcccctggcagcgagtacggcagcccgtcggtcatcagcgtcagcaaaggcagccctgacggcagccacccggtggtggtggcgccctacaacggcgggccgccgcgcacgtgccccaagatcaagcaggaggcggtctcttcgtgcacccacttgggcgctggaccccctctcagcaatggccaccggccggctgcacacgacttccccctggggcggcagctccccagcaggactaccccgaccctgggtcttgaggaagtgctgagcagcagggactgtcaccctgccctgccgcttcctcccggcttccatccccacccggggcccaattacccatccttcctgcccgatcagatgcagccgcaagtcccgccgctccattaccaagagctcatgccacccggttcctgcatgccagaggagcccaagccaaagaggggaagacgatcgtggccccggaaaaggaccgccacccacacttgtgattacgcgggctgcggcaaaacctacacaaagagttcccatctcaaggcacacctgcgaacccacacaggtgagaaaccttaccactgtgactgggacggctgtggatggaaattcgcccgctcagatgaactgaccaggcactaccgtaaacacacggggcaccgcccgttccagtgccaaaaatgcgaccgagcattttccaggtcggaccacctcgccttacacatgaagaggcatttt

SEQ ID NO: 45 - protein, 470 aa, Homo sapiens
MAVSDALLPSFSTFASGPAGREKTLRQAGAPNNRWREELSHMKRLPPVLPGRPYDLAAATVATDLESGGAGAACGGSNLAPLPRRETEEFNDLLDLDFILSNSLTHPPESVAATVSSSASASSSSSPSSSGPASAPSTCSFTYPIRAGNDPGVAPGGTGGGLLYGRESAPPPTAPFNLADINDVSPSGGFVAELLRPELDPVYIPPQQPQPPGGGLMGKFVLKASLSAPGSEYGSPSVISVSKGSPDGSHPVVVAPYNGGPPRTCPKIKQEAVSSCTHLGAGPPLSNGHRPAAHDFPLGRQLPSRTTPTLGLEEVLSSRDCHPALPLPPGFHPHPGPNYPSFLPDQMQPQVPPLHYQELMPPGSCMPEEPKPKRGRRSWPRKRTATHTCDYAGCGKTYTKSSHLKAHLRTHTGEKPYHCDWDGCGWKFARSDELTRHYRKHTGHRPFQCQKCDRAFSRSDHLALHMKRHF

SEQ ID NO: 46 - DNA, 235 bp, Artificial Sequence
  Synthetic Polynucleotide
attttaatctcactagggttctgggagcacccccccccaccgctcccgccctccacaaagctcctgggcccctcctcccttcaaggattgcgaagagctggtcgcaaatcctcctaagccaccagcatctcggtcttcagctcacaccagccttgagcccagcctgcggccaggggaccacgcacgtcccacccacccagcgactccccagccgctgcccactcttcctcactca

SEQ ID NO: 47 - DNA, 229 bp, Artificial Sequence
  Synthetic Polynucleotide
aatgtagtcttatgcaatactcttgtagtcttgcaacatggtaacgatgagttagcaacatgccttacaaggagagaaaaagcaccgtgcatgccgattggtggaagtaaggtggtacgatcgtgccttattaggaaggcaacagacgggtctgacatggattggacgaaccactgaattgccgcattgcagagatattgtatttaagtgcctagctcgatacataaac

SEQ ID NO: 48 - DNA, 617 bp, Artificial Sequence
  Synthetic Polynucleotide
cattgattattgactagttattaatagtaatcaattacggggtcattagttcatagcccatatatggagttccgcgttacataacttacggtaaatggcccgcctggctgaccgcccaacgacccccgcccattgacgtcaataatgacgtatgttcccatagtaacgccaatagggactttccattgacgtcaatgggtggactatttacggtaaactgcccacttggcagtacatcaagtgtatcatatgccaagtacgccccctattgacgtcaatgacggtaaatggcccgcctggcattatgcccagtacatgaccttatgggactttcctacttggcagtacatctacgtattagtcatcgctattaccatggtgatgcggttttggcagtacatcaatgggcgtggatagcggtttgactcacggggatttccaagtctccaccccattgacgtcaatgggagtttgttttggcaccaaaatcaacgggactttccaaaatgtcgtaacaactccgccccattgacgcaaatgggcggtaggcgtgtacggtgggaggtctatataagcagagctggtttagtgaaccgtcagatccgctagagatccgc

SEQ ID NO: 49 - DNA, 252 bp, Artificial Sequence
  Synthetic Polynucleotide
tcgagtggctccggtgcccgtcagtgggcagagcgcacatcgcccacagtccccgagaagttggggggaggggtcggcaattgaaccggtgcctagagaaggtggcgcggggtaaactgggaaagtgatgtcgtgtactggctccgcctttttcccgagggtgggggagaaccgtatataagtgcagtagtcgccgtgaacgttctttttcgcaacgggtttgccgccagaacacaggtgtcgtgaccgcgg

SEQ ID NO: 50 - DNA, 292 bp, Artificial Sequence
  Synthetic Polynucleotide
gggccccagaagcctggtggttgtttgtccttctcaggggaaaagtgaggcggccccttggaggaaggggccgggcagaatgatctaatcggattccaagcagctcaggggattgtctttttctagcaccttcttgccactcctaagcgtcctccgtgaccccggctgggatttcgcctggtgctgtgtcagccccggtctcccaggggcttcccagtggtccccaggaaccctcgacagggcccggtctctctcgtccagcaagggcagggacgggccacaggccaagggc

SEQ ID NO: 51 - DNA, 113 bp, Artificial Sequence
  Synthetic Polynucleotide
gcctgtagccttaatctctcctagcagggggtttgggggagggaggaggagaaagaaagggccccttatggctgagacacaatgacccagccacaaggagggattaccgggcg

SEQ ID NO: 52 - DNA, 281 bp, Artificial Sequence
  Synthetic Polynucleotide
aggtaggaagtggcctttaactccatagaccctatttaaacagcttcggacaggtttaaacatctccttggataattcctagtatccctgttcccactcctactcagggatgatagctctaagaggtgttaggggattaggctgaaaatgtaggtcacccctcagccatctgggaactagaatgagtgagagaggagagaggggcagagacacacacattcgcatattaaggtgacgcgtgtggcctcgaacaccgagcgaccctgcagcgacccgcttaa

SEQ ID NO: 53 - DNA, 26 bp, Artificial Sequence
  Synthetic Polynucleotide
aacgtatctacagtttactccctatc

SEQ ID NO: 54 - DNA, 21 bp, Artificial Sequence
  Synthetic Polynucleotide
ggtaggaagtggtacggaaag

SEQ ID NO: 55 - DNA, 20 bp, Artificial Sequence
  Synthetic Polynucleotide
cactgacaattccgtggtgt

SEQ ID NO: 56 - DNA, 20 bp, Artificial Sequence
  Synthetic Polynucleotide
gagatccgactcgtctgagg

SEQ ID NO: 57 - DNA, 20 bp, Artificial Sequence
  Synthetic Polynucleotide
tgggaagacaacctgtaggg

SEQ ID NO: 58 - DNA, 20 bp, Artificial Sequence
  Synthetic Polynucleotide
tgaaaccccgtctctaccaa

SEQ ID NO: 59 - DNA, 19 bp, Artificial Sequence
  Synthetic Polynucleotide
acatcgccaatcagcttgg

SEQ ID NO: 60 - DNA, 23 bp, Artificial Sequence
  Synthetic Polynucleotide
agaaccatactcgaaccacatcc

SEQ ID NO: 61 - DNA, 20 bp, Artificial Sequence
  Synthetic Polynucleotide
acagatgcaaccgatgcacc

SEQ ID NO: 62 - DNA, 20 bp, Artificial Sequence
  Synthetic Polynucleotide
tggagttgtactgcagggcg

SEQ ID NO: 63 - DNA, 19 bp, Artificial Sequence
  Synthetic Polynucleotide
gtgccccgactaaccgttg

SEQ ID NO: 64 - DNA, 20 bp, Artificial Sequence
  Synthetic Polynucleotide
gtcgttgaactcctcggtct

SEQ ID NO: 65 - DNA, 21 bp, Artificial Sequence
  Synthetic Polynucleotide
atgcccctcaacgtgaacttc

SEQ ID NO: 66 - DNA, 21 bp, Artificial Sequence
  Synthetic Polynucleotide
cgcaacataggatggagagca

SEQ ID NO: 67 - DNA, 22 bp, Artificial Sequence
  Synthetic Polynucleotide
gcgacaacaagaagacgcgcat

SEQ ID NO: 68 - DNA, 21 bp, Artificial Sequence
  Synthetic Polynucleotide
ctggatgttgggcaggacgcc

SEQ ID NO: 69 - DNA, 22 bp, Artificial Sequence
  Synthetic Polynucleotide
aagaaggacggcaagaagcgca

SEQ ID NO: 70 - DNA, 22 bp, Artificial Sequence
  Synthetic Polynucleotide
cgctcgaagatgtcgttcacga

SEQ ID NO: 71 - DNA, 21 bp, Artificial Sequence
  Synthetic Polynucleotide
gaagaagcctcaccgctaccg

SEQ ID NO: 72 - DNA, 23 bp, Artificial Sequence
  Synthetic Polynucleotide
ggttggtgtcctcaaacagaccc

SEQ ID NO: 73 - DNA, 22 bp, Artificial Sequence
  Synthetic Polynucleotide
aacatccagggcatcaccaagc

SEQ ID NO: 74 - DNA, 22 bp, Artificial Sequence
  Synthetic Polynucleotide
gttctccaggaacaccttcagc

SEQ ID NO: 75 - DNA, 19 bp, Artificial Sequence
  Synthetic Polynucleotide
ccggcctcaaggctctcta

SEQ ID NO: 76 - DNA, 20 bp, Artificial Sequence
  Synthetic Polynucleotide
tgccgcctcatactctcgaa

SEQ ID NO: 77 - DNA, 20 bp, Artificial Sequence
  Synthetic Polynucleotide
agtgtgacgttgacatccgt

SEQ ID NO: 78 - DNA, 20 bp, Artificial Sequence
  Synthetic Polynucleotide
tgctaggagccagagcagta

SEQ ID NO: 79 - DNA, 21 bp, Artificial Sequence
  Synthetic Polynucleotide
tcttcctggtccccacagttt

SEQ ID NO: 80 - DNA, 23 bp, Artificial Sequence
  Synthetic Polynucleotide
gcaagaatagttctcgggatgaa

SEQ ID NO: 81 - DNA, 25 bp, Artificial Sequence
  Synthetic Polynucleotide
gtgtcttcctcaactttctccttgg

SEQ ID NO: 82 - DNA, 26 bp, Artificial Sequence
  Synthetic Polynucleotide
cgcggacagccgcggccgtggattgc

SEQ ID NO: 83 - DNA, 27 bp, Artificial Sequence
  Synthetic Polynucleotide
ggctccttgctgtcattcatcttccac

SEQ ID NO: 84 - DNA, 26 bp, Artificial Sequence
  Synthetic Polynucleotide
caccgccgtcaggatctggaagttgg

SEQ ID NO: 85 - DNA, 19 bp, Artificial Sequence
  Synthetic Polynucleotide
ccggcctcaaggctctcta

SEQ ID NO: 86 - DNA, 20 bp, Artificial Sequence
  Synthetic Polynucleotide
tgccgcctcatactctcgaa

SEQ ID NO: 87 - DNA, 20 bp, Artificial Sequence
  Synthetic Polynucleotide
tcaagcaatggaccactggg

SEQ ID NO: 88 - DNA, 20 bp, Artificial Sequence
  Synthetic Polynucleotide
tctccatgagctccctgaca

SEQ ID NO: 89 - DNA, 22 bp, Artificial Sequence
  Synthetic Polynucleotide
actcctggtgaacaaagtcaga

SEQ ID NO: 90 - DNA, 20 bp, Artificial Sequence
  Synthetic Polynucleotide
catccctgagagctcttgcc

SEQ ID NO: 91 - DNA, 22 bp, Artificial Sequence
  Synthetic Polynucleotide
ccaatgtgtccgtcgtggatct

SEQ ID NO: 92 - DNA, 22 bp, Artificial Sequence
  Synthetic Polynucleotide
gttgaagtcgcaggagacaacc

SEQ ID NO: 93 - DNA, 23 bp, Artificial Sequence
  Synthetic Polynucleotide
acatcaagacatcgtgcgatatt

SEQ ID NO: 94 - DNA, 20 bp, Artificial Sequence
  Synthetic Polynucleotide
ccagcggtacacaaagacca

SEQ ID NO: 95 - DNA, 21 bp, Artificial Sequence
  Synthetic Polynucleotide
aagcacctccgaaagtacgtg

SEQ ID NO: 96 - DNA, 23 bp, Artificial Sequence
  Synthetic Polynucleotide
ctccagctctaccttacagttga

SEQ ID NO: 97 - DNA, 23 bp, Artificial Sequence
  Synthetic Polynucleotide
gatagaaccaaccatgttgaggg

SEQ ID NO: 98 - DNA, 21 bp, Artificial Sequence
  Synthetic Polynucleotide
tggagctttgtagccagaggt

SEQ ID NO: 99 - DNA, 22 bp, Artificial Sequence
  Synthetic Polynucleotide
caccattggcaatgagcggttc

SEQ ID NO: 100 - DNA, 22 bp, Artificial Sequence
  Synthetic Polynucleotide
aggtctttgcggatgtccacgt

SEQ ID NO: 101 - DNA, 492 bp, Homo sapiens
gatccggttccaggcctcggccctaaatagtctccctgggctttcaagagaaccacatgagaaaggaggattcgggctctgagcagtttcaccacccaccccccagtctgcaaatcctgacccgtgggtccacctgccccaaaggcggacgcaggacagtagaagggaacagagaacacataaacacagagagggccacagcggctcccacagtcaccgccaccttcctggcggggatgggtggggcgtctgagtttggttcccagcaaatccctctgagccgcccttgcgggctcgcctcaggagcaggggagcaagaggtgggaggaggaggtctaagtcccaggcccaattaagagatcaggtagtgtagggtttgggagcttttaaggtgaagaggcccgggctgatcccacaggccagtataaagcgccgtgaccctcaggtgatgcgccagggccggctgccgtcggggacagggctttccatagc

SEQ ID NO: 102 - DNA, 900 bp, Homo sapiens
agttaatgattaacccgccatgctacttatctacgtagccatgctctaggaagatcggaattcgcccttaagctagcagatcttccccacctagccacctggcaaactgctccttctctcaaaggcccaaacatggcctcccagactgcaacccccaggcagtcaggccctgtctccacaacctcacagccaccctggacggaatctgcttcttcccacatttgagtcctcctcagcccctgagctcctctgggcagggctgtttctttccatctttgtattcccaggggcctgcaaataaatgtttaatgaacgaacaagagagtgaattccaattccatgcaacaaggattgggctcctgggccctaggctatgtgtctggcaccagaaacggaagctgcaggttgcagcccctgccctcatggagctcctcctgtcagaggagtgtggggactggatgactccagaggtaacttgtgggggaacgaacaggtaaggggctgtgtgacgagatgagagactgggagaataaaccagaaagtctctagctgtccagaggacatagcacagaggcccatggtccctatttcaaacccaggccaccagactgagctgggaccttgggacagacaagtcatgcagaagttaggggaccttctcctcccttttcctggatggatcctgagtaccttctcctccctgacctcaggcttcctcctagtgtcaccttggcccctcttagaagccaattaggccctcagtttctgcagcggggattaatatgattatgaacacccccaatctcccagatgctgattcagccaggagcttaggagggggaggtcactttataagggtctgggggggtcagaacccagagtcatcccctgaattctgca

SEQ ID NO: 103 - DNA, 521 bp, Mus musculus
ggttcttcccattttggctacatggtctttttttttacctttttggttcctttggccttttggcttttggcttccagggcttctggatcccccccaacccctcccatacacatacacatgtgcactcgtgcactcaacccagcacaggataatgttcattcttgacctttccacatacatctggctatgttctctctcttatctacaataaatctcctccactatacttaggagcagttatgttcttcttctttctttcttttttttttttttcattcagtaacatcatcagaatcccctagctctggcctacctcctcagtaacaatcagctgatccctggccactaatctgtactcactaatctgttttccaaactcttggcccctgagctaattatagcagtgcttcatgccacccaccccaaccctattcttgttctctgactcccactaatctacacattcagaggattgtggatataagaggctgggaggccagcttagcaaccagagctggagg

SEQ ID NO: 104 - DNA, 292 bp, Homo sapiens
gggccccagaagcctggtggttgtttgtccttctcaggggaaaagtgaggcggccccttggaggaaggggccgggcagaatgatctaatcggattccaagcagctcaggggattgtctttttctagcaccttcttgccactcctaagcgtcctccgtgaccccggctgggatttagcctggtgctgtgtcagccccggtctcccaggggcttcccagtggtccccaggaaccctcgacagggcccggtctctctcgtccagcaagggcagggacgggccacaggccaagggc

SEQ ID NO: 105 - DNA, 7390 bp, Homo sapiens
ttatgcagtgctgccataaccatgagtgataacactgcggccaacttacttctgacaacgatcggaggaccgaaggagctaaccgcttttttgcacaacatgggggatcatgtaactcgccttgatcgttgggaaccggagctgaatgaagccataccaaacgacgagcgtgacaccacgatgcctgtagtaatggtaacaacgttgcgcaaactattaactggcgaactacttactctagcttcccggcaacaattaatagactggatggaggcggataaagttgcaggaccacttctgcgctcggcccttccggctggctggtttattgctgataaatctggagccggtgagcgtgggtctcgcggtatcattgcagcactggggccagatggtaagccctcccgtatcgtagttatctacacgacggggagtcaggcaactatggatgaacgaaatagacagatcgctgagataggtgcctcactgattaagcattggtaactgtcagaccaagtttactcatatatactttagattgatttaaaacttcatttttaatttaaaaggatctaggtgaagatcctttttgataatctcatgaccaaaatcccttaacgtgagttttcgttccactgagcgtcagaccccgtagaaaagatcaaaggatcttcttgagatcctttttttctgcgcgtaatctgctgcttgcaaacaaaaaaaccaccgctaccagcggtggtttgtttgccggatcaagagctaccaactctttttccgaaggtaactggcttcagcagagcgcagataccaaatactgtccttctagtgtagccgtagttaggccaccacttcaagaactctgtagcaccgcctacatacctcgctctgctaatcctgttaccagtggctgctgccagtggcgataagtcgtgtcttaccgggttggactcaagacgatagttaccggataaggcgcagcggtcgggctgaacggggggttcgtgcacacagcccagcttggagcgaacgacctacaccgaactgagatacctacagcgtgagctatgagaaagcgccacgcttcccgaagggagaaaggcggacaggtatccggtaagcggcagggtcggaacaggagagcgcacgagggagcttccagggggaaacgcctggtatctttatagtcctgtcgggtttcgccacctctgacttgagcgtcgatttttgtgatgctcgtcaggggggcggagcctatggaaaaacgccagcaacgcggcctttttacggttcctggccttttgctggccttttgctcacatgttctttcctgcgttatcccctgattctgtggataaccgtattaccgcctttgagtgagctgataccgctcgccgcagccgaacgaccgagcgcagcgagtcagtgagcgaggaagcggaagagcgcccaatacgcaaaccgcctctccccgcgcgttggccgattcattaatgcagctggcacgacaggtttcccgactggaaagcgggcagtgagcgcaacgcaattaatgtgagttagctcactcattaggcaccccaggctttacactttatgcttccggctcgtatgttgtgtggaattgtgagcggataacaatttcacacaggaaacagctatgaccatgattacgccagatttaattaaggccttaattaggctgcgcgctcgctcgctcactgaggccgcccgggcaaagcccgggcgtcgggcgacctttggtcgcccggcctcagtgagcgagcgagcgcgcagagagggagtggccaactccatcactaggggttccttgtagttaatgattaacccgccatgctacttatctacgtagccatgctctaggaagatcggaattctttactccctatcagtgatagagaacgtatgaagagtttactccctatcagtgatagagaacgtatgcagactttactccctatcagtgatagagaacgtataaggagtttactccctatcagtgatagagaacgtatgaccagtttactccctatcagtgatagagaacgtatctacagtttactccctatcagtgatagagaacgtatatccagtttactccctatcagtgatagagaacgtataagctttaggcgtgtacggtgggcgcctataaaagcagagctcgtttagtgaaccgtcagatcgcctggagcaattccacaacacttttgtcttataccaactttccgtaccacttcctaccctcgtaaagcggccgcgccaccatggcgggacacctggcttcggatttcgccttctcgccccctccaggtggtggaggtgatgggccaggggggccggagccgggctgggttgatcctcggacctggctaagcttccaaggccctcctggagggccaggaatcgggccgggggttgggccaggctctgaggtgtgggggattcccccatgccccccgccgtatgagttctgtggggggatggcgtactgtgggccccaggttggagtggggctagtgccccaaggcggcttggagacctctcagcctgagggcgaagcaggagtcggggtggagagcaactccgatggggcctccccggagccctgcaccgtcacccctggtgccgtgaagctggagaaggagaagctggagcaaaacccggaggagtcccaggacatcaaagctctgcagaaagaactcgagcaatttgccaagctcctgaagcagaagaggatcaccctgggatatacacaggccgatgtggggctcaccctgggggttctatttgggaaggtattcagccaaacgaccatctgccgctttgaggctctgcagcttagcttcaagaacatgtgtaagctgcggcccttgctgcagaagtgggtggaggaagctgacaacaatgaaaatcttcaggagatatgcaaagcagaaaccctcgtgcaggcccgaaagagaaagcgaaccagtatcgagaaccgagtgagaggcaacctggagaatttgttcctgcagtgcccgaaacccacactgcagcagatcagccacatcgcccagcagcttgggctcgagaaggatgtggtccgagtgtggttctgtaaccggcgccagaagggcaagcgatcaagcagcgactatgcacaacgagaggattttgaggctgctgggtctcctttctcagggggaccagtgtcctttcctctggccccagggccccattttggtaccccaggctatgggagccctcacttcactgcactgtactcctcggtccctttccctgagggggaagcctttccccctgtctctgtcaccactctgggctctcccatgcattcaaacgctagcggcagcggcgccacgaacttctctctgttaaagcaagcaggagatgttgaagaaaaccccgggcctgcatgcatgtacaacatgatggagacggagctgaagccgccgggcccgcagcaaacttcggggggcggcggcggcaactccaccgcggcggcggccggcggcaaccagaaaaacagcccggaccgcgtcaagcggcccatgaatgccttcatggtgtggtcccgcgggcagcggcgcaagatggcccaggagaaccccaagatgcacaactcggagatcagcaagcgcctgggcgccgagtggaaacttttgtcggagacggagaagcggccgttcatcgacgaggctaagcggctgcgagcgctgcacatgaaggagcacccggattataaataccggccccggcggaaaaccaagacgctcatgaagaaggataagtacacgctgcccggcgggctgctggcccccggcggcaatagcatggcgagcggggtcggggtgggcgccggcctgggcgcgggcgtgaaccagcgcatggacagttacgcgcacatgaacggctggagcaacggcagctacagcatgatgcaggaccagctgggctacccgcagcacccgggcctcaatgcgcacggcgcagcgcagatgcagcccatgcaccgctacgacgtgagcgccctgcagtacaactccatgaccagctcgcagacctacatgaacggctcgcccacctacagcatgtcctactcgcagcagggcacccctggcatggctcttggctccatgggttcggtggtcaagtccgaggccagctccagcccccctgtggttacctcttcctcccactccagggcgccctgccaggccggggacctccgggacatgatcagcatgtatctccccggcgccgaggtgccggaacccgccgcccccagcagacttcacatgtcccagcactaccagagcggcccggtgcccggcacggccattaacggcacactgcccctctcacacatggcatgcggctccggcgagggcaggggaagtcttctaacatgcggggacgtggaggaaaatcccggcccactcgagatggctgtcagcgacgcgctgctcccatctttctccacgttcgcgtctggcccggcgggaagggagaagacactgcgtcaagcaggtgccccgaataaccgctggcgggaggagctctcccacatgaagcgacttcccccagtgcttcccggccgcccctatgacctggcggcggcgaccgtggccacagacctggagagcggcggagccggtgcggcttgcggcggtagcaacctggcgcccctacctcggagagagaccgaggagttcaacgatctcctggacctggactttattctctccaattcgctgacccatcctccggagtcagtggccgccaccgtgtcctcgtcagcgtcagcctcctcttcgtcgtcgccgtcgagcagcggccctgccagcgcgccctccacctgcagcttcacctatccgatccgggccgggaacgacccgggcgtggcgccgggcggcacgggcggaggcctcctctatggcagggagtccgctccccctccgacggctcccttcaacctggcggacatcaacgacgtgagcccctcgggcggcttcgtggccgagctcctgcggccagaattggacccggtgtacattccgccgcagcagccgcagccgccaggtggcgggctgatgggcaagttcgtgctgaaggcgtcgctgagcgcccctggcagcgagtacggcagcccgtcggtcatcagcgtcagcaaaggcagccctgacggcagccacccggtggtggtggcgccctacaacggcgggccgccgcgcacgtgccccaagatcaagcaggaggcggtctcttcgtgcacccacttgggcgctggaccccctctcagcaatggccaccggccggctgcacacgacttccccctggggcggcagctccccagcaggactaccccgaccctgggtcttgaggaagtgctgagcagcagggactgtcaccctgccctgccgcttcctcccggcttccatccccacccggggcccaattacccatccttcctgcccgatcagatgcagccgcaagtcccgccgctccattaccaagagctcatgccacccggttcctgcatgccagaggagcccaagccaaagaggggaagacgatcgtggccccggaaaaggaccgccacccacacttgtgattacgcgggctgcggcaaaacctacacaaagagttcccatctcaaggcacacctgcgaacccacacaggtgagaaaccttaccactgtgactgggacggctgtggatggaaattcgcccgctcagatgaactgaccaggcactaccgtaaacacacggggcaccgcccgttccagtgccaaaaatgcgaccgagcattttccaggtcggaccacctcgccttacacatgaagaggcatttttaaatgactagtgcgcgcagcggccgaccatggcccaacttgtttattgcagcttataatggttacaaataaagcaatagcatcacaaatttcacaaataaagcatttttttcactgcattctagttgtggtttgtccaaactcatcaatgtatcttatcatgtctggatctcggtaccggatccaaattcccgataaggatcttcctagagcatggctacgtagataagtagcatggcgggttaatcattaactacaaggaacccctagtgatggagttggccactccctctctgcgcgctcgctcgctcactgaggccgggcgaccaaaggtcgcccgacgcccgggctttgcccgggcggcctcagtgagcgagcgagcgcgcagccttaattaacctaattcactggccgtcgttttacaacgtcgtgactgggaaaaccctggcgttacccaacttaatcgccttgcagcacatccccctttcgccagctggcgtaatagcgaagaggcccgcaccgatcgcccttcccaacagttgcgcagcctgaatggcgaatgggacgcgccctgtagcggcgcattaagcgcggcgggtgtggtggttacgcgcagcgtgaccgctacacttgccagcgccctagcgcccgctcctttcgctttcttcccttcctttctcgccacgttcgccggctttccccgtcaagctctaaatcgggggctccctttagggttccgatttagtgctttacggcacctcgaccccaaaaaacttgattagggtgatggttcacgtagtgggccatcgccctgatagacggtttttcgccctttgacgttggagtccacgttctttaatagtggactcttgttccaaactggaacaacactcaaccctatctcggtctattcttttgatttataagggattttgccgatttcggcctattggttaaaaaatgagctgatttaacaaaaatttaacgcgaattttaacaaaatattaacgtttataatttcaggtggcatctttcggggaaatgtgcgcggaacccctatttgtttatttttctaaatacattcaaatatgtatccgctcatgagacaataaccctgataaatgcttcaataatattgaaaaaggaagagtatgagtattcaacatttccgtgtcgcccttattcccttttttgcggcattttgccttcctgtttttgctcacccagaaacgctggtgaaagtaaaagatgctgaagatcagttgggtgcacgagtgggttacatcgaactggatctcaatagtggtaagatccttgagagttttcgccccgaagaacgttttccaatgatgagcacttttaaagttctgctatgtggcgcggtattatcccgtattgacgccgggcaagagcaactcggtcgccgcatacactattctcagaatgacttggttgagtactcaccagtcacagaaaagcatcttacggatggcatgacagtaagagaa

SEQ ID NO: 106 - DNA, 7265 bp, Homo sapiens
ttatgcagtgctgccataaccatgagtgataacactgcggccaacttacttctgacaacgatcggaggaccgaaggagctaaccgcttttttgcacaacatgggggatcatgtaactcgccttgatcgttgggaaccggagctgaatgaagccataccaaacgacgagcgtgacaccacgatgcctgtagtaatggtaacaacgttgcgcaaactattaactggcgaactacttactctagcttcccggcaacaattaatagactggatggaggcggataaagttgcaggaccacttctgcgctcggcccttccggctggctggtttattgctgataaatctggagccggtgagcgtgggtctcgcggtatcattgcagcactggggccagatggtaagccctcccgtatcgtagttatctacacgacggggagtcaggcaactatggatgaacgaaatagacagatcgctgagataggtgcctcactgattaagcattggtaactgtcagaccaagtttactcatatatactttagattgatttaaaacttcatttttaatttaaaaggatctaggtgaagatcctttttgataatctcatgaccaaaatcccttaacgtgagttttcgttccactgagcgtcagaccccgtagaaaagatcaaaggatcttcttgagatcctttttttctgcgcgtaatctgctgcttgcaaacaaaaaaaccaccgctaccagcggtggtttgtttgccggatcaagagctaccaactctttttccgaaggtaactggcttcagcagagcgcagataccaaatactgtccttctagtgtagccgtagttaggccaccacttcaagaactctgtagcaccgcctacatacctcgctctgctaatcctgttaccagtggctgctgccagtggcgataagtcgtgtcttaccgggttggactcaagacgatagttaccggataaggcgcagcggtcgggctgaacggggggttcgtgcacacagcccagcttggagcgaacgacctacaccgaactgagatacctacagcgtgagctatgagaaagcgccacgcttcccgaagggagaaaggcggacaggtatccggtaagcggcagggtcggaacaggagagcgcacgagggagcttccagggggaaacgcctggtatctttatagtcctgtcgggtttcgccacctctgacttgagcgtcgatttttgtgatgctcgtcaggggggcggagcctatggaaaaacgccagcaacgcggcctttttacggttcctggccttttgctggccttttgctcacatgttctttcctgcgttatcccctgattctgtggataaccgtattaccgcctttgagtgagctgataccgctcgccgcagccgaacgaccgagcgcagcgagtcagtgagcgaggaagcggaagagcgcccaatacgcaaaccgcctctccccgcgcgttggccgattcattaatgcagctggcacgacaggtttcccgactggaaagcgggcagtgagcgcaacgcaattaatgtgagttagctcactcattaggcaccccaggctttacactttatgcttccggctcgtatgttgtgtggaattgtgagcggataacaatttcacacaggaaacagctatgaccatgattacgccagatttaattaaggccttaattaggctgcgcgctcgctcgctcactgaggccgcccgggcaaagcccgggcgtcgggcgacctttggtcgcccggcctcagtgagcgagcgagcgcgcagagagggagtggccaactccatcactaggggttccttgtagttaatgattaacccgccatgctacttatctacgtagccatgctctaggaagatcggaattctcgagtggctccggtgcccgtcagtgggcagagcgcacatcgcccacagtccccgagaagttggggggaggggtcggcaattgaaccggtgcctagagaaggtggcgcggggtaaactgggaaagtgatgtcgtgtactggctccgcctttttcccgagggtgggggagaaccgtatataagtgcagtagtcgccgtgaacgttctttttcgcaacgggtttgccgccagaacacaggtgtcgtgacgcgggcggccgcgccaccatggcgggacacctggcttcggatttcgccttctcgccccctccaggtggtggaggtgatgggccaggggggccggagccgggctgggttgatcctcggacctggctaagcttccaaggccctcctggagggccaggaatcgggccgggggttgggccaggctctgaggtgtgggggattcccccatgccccccgccgtatgagttctgtggggggatggcgtactgtgggccccaggttggagtggggctagtgccccaaggcggcttggagacctctcagcctgagggcgaagcaggagtcggggtggagagcaactccgatggggcctccccggagccctgcaccgtcacccctggtgccgtgaagctggagaaggagaagctggagcaaaacccggaggagtcccaggacatcaaagctctgcagaaagaactcgagcaatttgccaagctcctgaagcagaagaggatcaccctgggatatacacaggccgatgtggggctcaccctgggggttctatttgggaaggtattcagccaaacgaccatctgccgctttgaggctctgcagcttagcttcaagaacatgtgtaagctgcggcccttgctgcagaagtgggtggaggaagctgacaacaatgaaaatcttcaggagatatgcaaagcagaaaccctcgtgcaggcccgaaagagaaagcgaaccagtatcgagaaccgagtgagaggcaacctggagaatttgttcctgcagtgcccgaaacccacactgcagcagatcagccacatcgcccagcagcttgggctcgagaaggatgtggtccgagtgtggttctgtaaccggcgccagaagggcaagcgatcaagcagcgactatgcacaacgagaggattttgaggctgctgggtctcctttctcagggggaccagtgtcctttcctctggccccagggccccattttggtaccccaggctatgggagccctcacttcactgcactgtactcctcggtccctttccctgagggggaagcctttccccctgtctctgtcaccactctgggctctcccatgcattcaaacgctagcggcagcggcgccacgaacttctctctgttaaagcaagcaggagatgttgaagaaaaccccgggcctgcatgcatgtacaacatgatggagacggagctgaagccgccgggcccgcagcaaacttcggggggcggcggcggcaactccaccgcggcggcggccggcggcaaccagaaaaacagcccggaccgcgtcaagcggcccatgaatgccttcatggtgtggtcccgcgggcagcggcgcaagatggcccaggagaaccccaagatgcacaactcggagatcagcaagcgcctgggcgccgagtggaaacttttgtcggagacggagaagcggccgttcatcgacgaggctaagcggctgcgagcgctgcacatgaaggagcacccggattataaataccggccccggcggaaaaccaagacgctcatgaagaaggataagtacacgctgcccggcgggctgctggcccccggcggcaatagcatggcgagcggggtcggggtgggcgccggcctgggcgcgggcgtgaaccagcgcatggacagttacgcgcacatgaacggctggagcaacggcagctacagcatgatgcaggaccagctgggctacccgcagcacccgggcctcaatgcgcacggcgcagcgcagatgcagcccatgcaccgctacgacgtgagcgccctgcagtacaactccatgaccagctcgcagacctacatgaacggctcgcccacctacagcatgtcctactcgcagcagggcacccctggcatggctcttggctccatgggttcggtggtcaagtccgaggccagctccagcccccctgtggttacctcttcctcccactccagggcgccctgccaggccggggacctccgggacatgatcagcatgtatctccccggcgccgaggtgccggaacccgccgcccccagcagacttcacatgtcccagcactaccagagcggcccggtgcccggcacggccattaacggcacactgcccctctcacacatggcatgcggctccggcgagggcaggggaagtcttctaacatgcggggacgtggaggaaaatcccggcccactcgagatggctgtcagcgacgcgctgctcccatctttctccacgttcgcgtctggcccggcgggaagggagaagacactgcgtcaagcaggtgccccgaataaccgctggcgggaggagctctcccacatgaagcgacttcccccagtgcttcccggccgcccctatgacctggcggcggcgaccgtggccacagacctggagagcggcggagccggtgcggcttgcggcggtagcaacctggcgcccctacctcggagagagaccgaggagttcaacgatctcctggacctggactttattctctccaattcgctgacccatcctccggagtcagtggccgccaccgtgtcctcgtcagcgtcagcctcctcttcgtcgtcgccgtcgagcagcggccctgccagcgcgccctccacctgcagcttcacctatccgatccgggccgggaacgacccgggcgtggcgccgggcggcacgggcggaggcctcctctatggcagggagtccgctccccctccgacggctcccttcaacctggcggacatcaacgacgtgagcccctcgggcggcttcgtggccgagctcctgcggccagaattggacccggtgtacattccgccgcagcagccgcagccgccaggtggcgggctgatgggcaagttcgtgctgaaggcgtcgctgagcgcccctggcagcgagtacggcagcccgtcggtcatcagcgtcagcaaaggcagccctgacggcagccacccggtggtggtggcgccctacaacggcgggccgccgcgcacgtgccccaagatcaagcaggaggcggtctcttcgtgcacccacttgggcgctggaccccctctcagcaatggccaccggccggctgcacacgacttccccctggggcggcagctccccagcaggactaccccgaccctgggtcttgaggaagtgctgagcagcagggactgtcaccctgccctgccgcttcctcccggcttccatccccacccggggcccaattacccatccttcctgcccgatcagatgcagccgcaagtcccgccgctccattaccaagagctcatgccacccggttcctgcatgccagaggagcccaagccaaagaggggaagacgatcgtggccccggaaaaggaccgccacccacacttgtgattacgcgggctgcggcaaaacctacacaaagagttcccatctcaaggcacacctgcgaacccacacaggtgagaaaccttaccactgtgactgggacggctgtggatggaaattcgcccgctcagatgaactgaccaggcactaccgtaaacacacggggcaccgcccgttccagtgccaaaaatgcgaccgagcattttccaggtcggaccacctcgccttacacatgaagaggcatttttaaatgactagtgcgcgcagcggccgaccatggcccaacttgtttattgcagcttataatggttacaaataaagcaatagcatcacaaatttcacaaataaagcatttttttcactgcattctagttgtggtttgtccaaactcatcaatgtatcttatcatgtctggatctcggtaccggatccaaattcccgataaggatcttcctagagcatggctacgtagataagtagcatggcgggttaatcattaactacaaggaacccctagtgatggagttggccactccctctctgcgcgctcgctcgctcactgaggccgggcgaccaaaggtcgcccgacgcccgggctttgcccgggcggcctcagtgagcgagcgagcgcgcagccttaattaacctaattcactggccgtcgttttacaacgtcgtgactgggaaaaccctggcgttacccaacttaatcgccttgcagcacatccccctttcgccagctggcgtaatagcgaagaggcccgcaccgatcgcccttcccaacagttgcgcagcctgaatggcgaatgggacgcgccctgtagcggcgcattaagcgcggcgggtgtggtggttacgcgcagcgtgaccgctacacttgccagcgccctagcgcccgctcctttcgctttcttcccttcctttctcgccacgttcgccggctttccccgtcaagctctaaatcgggggctccctttagggttccgatttagtgctttacggcacctcgaccccaaaaaacttgattagggtgatggttcacgtagtgggccatcgccctgatagacggtttttcgccctttgacgttggagtccacgttctttaatagtggactcttgttccaaactggaacaacactcaaccctatctcggtctattcttttgatttataagggattttgccgatttcggcctattggttaaaaaatgagctgatttaacaaaaatttaacgcgaattttaacaaaatattaacgtttataatttcaggtggcatctttcggggaaatgtgcgcggaacccctatttgtttatttttctaaatacattcaaatatgtatccgctcatgagacaataaccctgataaatgcttcaataatattgaaaaaggaagagtatgagtattcaacatttccgtgtcgcccttattcccttttttgcggcattttgccttcctgtttttgctcacccagaaacgctggtgaaagtaaaagatgctgaagatcagttgggtgcacgagtgggttacatcgaactggatctcaatagtggtaagatccttgagagttttcgccccgaagaacgttttccaatgatgagcacttttaaagttctgctatgtggcgcggtattatcccgtattgacgccgggcaagagcaactcggtcgccgcatacactattctcagaatgacttggttgagtactcaccagtcacagaaaagcatcttacggatggcatgacagtaagagaa

SEQ ID NO: 107 - DNA, 5437 bp, Artificial Sequence
  Synthetic Polynucleotide
ttatgcagtgctgccataaccatgagtgataacactgcggccaacttacttctgacaacgatcggaggaccgaaggagctaaccgcttttttgcacaacatgggggatcatgtaactcgccttgatcgttgggaaccggagctgaatgaagccataccaaacgacgagcgtgacaccacgatgcctgtagtaatggtaacaacgttgcgcaaactattaactggcgaactacttactctagcttcccggcaacaattaatagactggatggaggcggataaagttgcaggaccacttctgcgctcggcccttccggctggctggtttattgctgataaatctggagccggtgagcgtgggtctcgcggtatcattgcagcactggggccagatggtaagccctcccgtatcgtagttatctacacgacggggagtcaggcaactatggatgaacgaaatagacagatcgctgagataggtgcctcactgattaagcattggtaactgtcagaccaagtttactcatatatactttagattgatttaaaacttcatttttaatttaaaaggatctaggtgaagatcctttttgataatctcatgaccaaaatcccttaacgtgagttttcgttccactgagcgtcagaccccgtagaaaagatcaaaggatcttcttgagatcctttttttctgcgcgtaatctgctgcttgcaaacaaaaaaaccaccgctaccagcggtggtttgtttgccggatcaagagctaccaactctttttccgaaggtaactggcttcagcagagcgcagataccaaatactgtccttctagtgtagccgtagttaggccaccacttcaagaactctgtagcaccgcctacatacctcgctctgctaatcctgttaccagtggctgctgccagtggcgataagtcgtgtcttaccgggttggactcaagacgatagttaccggataaggcgcagcggtcgggctgaacggggggttcgtgcacacagcccagcttggagcgaacgacctacaccgaactgagatacctacagcgtgagctatgagaaagcgccacgcttcccgaagggagaaaggcggacaggtatccggtaagcggcagggtcggaacaggagagcgcacgagggagcttccagggggaaacgcctggtatctttatagtcctgtcgggtttcgccacctctgacttgagcgtcgatttttgtgatgctcgtcaggggggcggagcctatggaaaaacgccagcaacgcggcctttttacggttcctggccttttgctggccttttgctcacatgttctttcctgcgttatcccctgattctgtggataaccgtattaccgcctttgagtgagctgataccgctcgccgcagccgaacgaccgagcgcagcgagtcagtgagcgaggaagcggaagagcgcccaatacgcaaaccgcctctccccgcgcgttggccgattcattaatgcagctggcacgacaggtttcccgactggaaagcgggcagtgagcgcaacgcaattaatgtgagttagctcactcattaggcaccccaggctttacactttatgcttccggctcgtatgttgtgtggaattgtgagcggataacaatttcacacaggaaacagctatgaccatgattacgccagatttaattaaggccttaattaggctgcgcgctcgctcgctcactgaggccgcccgggcaaagcccgggcgtcgggcgacctttggtcgcccggcctcagtgagcgagcgagcgcgcagagagggagtggccaactccatcactaggggttccttgtagttaatgattaacccgccatgctacttatctacgtagccatgctctaggaagatcggaattctttactccctatcagtgatagagaacgtatgaagagtttactccctatcagtgatagagaacgtatgcagactttactccctatcagtgatagagaacgtataaggagtttactccctatcagtgatagagaacgtatgaccagtttactccctatcagtgatagagaacgtatctacagtttactccctatcagtgatagagaacgtatatccagtttactccctatcagtgatagagaacgtataagctttaggcgtgtacggtgggcgcctataaaagcagagctcgtttagtgaaccgtcagatcgcctggagcaattccacaacacttttgtcttataccaactttccgtaccacttcctaccctcgtaaagcggccgcatggaagacgccaaaaacataaagaaaggcccggcgccattctatccgctggaagatggaaccgctggagagcaactgcataaggctatgaagagatacgccctggttcctggaacaattgcttttacagatgcacatatcgaggtggacatcacttacgctgagtacttcgaaatgtccgttcggttggcagaagctatgaaacgatatgggctgaatacaaatcacagaatcgtcgtatgcagtgaaaactctcttcaattctttatgccggtgttgggcgcgttatttatcggagttgcagttgcgcccgcgaacgacatttataatgaacgtgaattgctcaacagtatgggcatttcgcagcctaccgtggtgttcgtttccaaaaaggggttgcaaaaaattttgaacgtgcaaaaaaagctcccaatcatccaaaaaattattatcatggattctaaaacggattaccagggatttcagtcgatgtacacgttcgtcacatctcatctacctcccggttttaatgaatacgattttgtgccagagtccttcgatagggacaagacaattgcactgatcatgaactcctctggatctactggtctgcctaaaggtgtcgctctgcctcatagaactgcctgcgtgagattctcgcatgccagagatcctatttttggcaatcaaatcattccggatactgcgattttaagtgttgttccattccatcacggttttggaatgtttactacactcggatatttgatatgtggatttcgagtcgtcttaatgtatagatttgaagaagagctgtttctgaggagccttcaggattacaagattcaaagtgcgctgctggtgccaaccctattctccttcttcgccaaaagcactctgattgacaaatacgatttatctaatttacacgaaattgcttctggtggcgctcccctctctaaggaagtcggggaagcggttgccaagaggttccatctgccaggtatcaggcaaggatatgggctcactgagactacatcagctattctgattacacccgagggggatgataaaccgggcgcggtcggtaaagttgttccattttttgaagcgaaggttgtggatctggataccgggaaaacgctgggcgttaatcaaagaggcgaactgtgtgtgagaggtcctatgattatgtccggttatgtaaacaatccggaagcgaccaacgccttgattgacaaggatggatggctacattctggagacatagcttactgggacgaagacgaacacttcttcatcgttgaccgcctgaagtctctgattaagtacaaaggctatcaggtggctcccgctgaattggaatccatcttgctccaacaccccaacatcttcgacgcaggtgtcgcaggtcttcccgacgatgacgccggtgaacttcccgccgccgttgttgttttggagcacggaaagacgatgacggaaaaagagatcgtggattacgtcgccagtcaagtaacaaccgcgaaaaagttgcgcggaggagttgtgtttgtggacgaagtaccgaaaggtcttaccggaaaactcgacgcaagaaaaatcagagagatcctcataaaggccaagaagggcggaaagatcgccgtgtaaactagtgcgcgcagcggccgaccatggcccaacttgtttattgcagcttataatggttacaaataaagcaatagcatcacaaatttcacaaataaagcatttttttcactgcattctagttgtggtttgtccaaactcatcaatgtatcttatcatgtctggatctcggtaccggatccaaattcccgataaggatcttcctagagcatggctacgtagataagtagcatggcgggttaatcattaactacaaggaacccctagtgatggagttggccactccctctctgcgcgctcgctcgctcactgaggccgggcgaccaaaggtcgcccgacgcccgggctttgcccgggcggcctcagtgagcgagcgagcgcgcagccttaattaacctaattcactggccgtcgttttacaacgtcgtgactgggaaaaccctggcgttacccaacttaatcgccttgcagcacatccccctttcgccagctggcgtaatagcgaagaggcccgcaccgatcgcccttcccaacagttgcgcagcctgaatggcgaatgggacgcgccctgtagcggcgcattaagcgcggcgggtgtggtggttacgcgcagcgtgaccgctacacttgccagcgccctagcgcccgctcctttcgctttcttcccttcctttctcgccacgttcgccggctttccccgtcaagctctaaatcgggggctccctttagggttccgatttagtgctttacggcacctcgaccccaaaaaacttgattagggtgatggttcacgtagtgggccatcgccctgatagacggtttttcgccctttgacgttggagtccacgttctttaatagtggactcttgttccaaactggaacaacactcaaccctatctcggtctattcttttgatttataagggattttgccgatttcggcctattggttaaaaaatgagctgatttaacaaaaatttaacgcgaattttaacaaaatattaacgtttataatttcaggtggcatctttcggggaaatgtgcgcggaacccctatttgtttatttttctaaatacattcaaatatgtatccgctcatgagacaataaccctgataaatgcttcaataatattgaaaaaggaagagtatgagtattcaacatttccgtgtcgcccttattcccttttttgcggcattttgccttcctgtttttgctcacccagaaacgctggtgaaagtaaaagatgctgaagatcagttgggtgcacgagtgggttacatcgaactggatctcaatagtggtaagatccttgagagttttcgccccgaagaacgttttccaatgatgagcacttttaaagttctgctatgtggcgcggtattatcccgtattgacgccgggcaagagcaactcggtcgccgcatacactattctcagaatgacttggttgagtactcaccagtcacagaaaagcatcttacggatggcatgacagtaagagaa

SEQ ID NO: 108 - DNA, 19 bp, Artificial Sequence
  Synthetic Polynucleotide
cacaagtcaaacctttatt

SEQ ID NO: 109 - DNA, 21 bp, Artificial Sequence
  Synthetic Polynucleotide
ggacgtaatccagaaagaaga

SEQ ID NO: 110 - DNA, 21 bp, Artificial Sequence
  Synthetic Polynucleotide
ttgtgcctctggaggttataa

SEQ ID NO: 111 - DNA, 21 bp, Artificial Sequence
  Synthetic Polynucleotide
ggaaataaaggctggtgaagg

SEQ ID NO: 112 - DNA, 21 bp, Artificial Sequence
  Synthetic Polynucleotide
gaaagatgaaggtccatatta

SEQ ID NO: 113 - DNA, 21 bp, Artificial Sequence
  Synthetic Polynucleotide
gcagatggccgtgacacaaat

SEQ ID NO: 114 - DNA, 21 bp, Artificial Sequence
  Synthetic Polynucleotide
gctcatggagactaggtttgg

SEQ ID NO: 115 - DNA, 21 bp, Artificial Sequence
  Synthetic Polynucleotide
ggatgtaagtttgccagaagc

SEQ ID NO: 116 - DNA, 21 bp, Artificial Sequence
  Synthetic Polynucleotide
gctccaacgagaagctatttg

SEQ ID NO: 117 - DNA, 19 bp, Artificial Sequence
  Synthetic Polynucleotide
gttcagatgtgcggcgagt

SEQ ID NO: 118 - protein, 22 aa, Artificial Sequence
  Synthetic Polypeptide
GSGATNFSLLKQAGDVEENPGP

SEQ ID NO: 119 - DNA, 66 bp, Artificial Sequence
  Synthetic Polynucleotide
ggcagcggcgccacgaacttctctctgttaaagcaagcaggagatgttgaagaaaaccccgggcct

SEQ ID NO: 120 - DNA, 63 bp, Artificial Sequence
  Synthetic Polynucleotide
ggctccggcgagggcaggggaagtcttctaacatgcggggacgtggaggaaaatcccggccca

SEQ ID NO: 121 - DNA, 7390 bp, Artificial Sequence; identical to SEQ ID NO: 105
  Synthetic Polynucleotide

SEQ ID NO: 122 - DNA, 6586 bp, Artificial Sequence
  Synthetic polynucleotide
aattcagagaccgggaaccaaactagcctttaaaaaacataagtacaggagccagcaagatggctcagtgggtaaaggtgcctaccagcaagcctgacagcctgagttcagtccccacgaactacgtggtaggagaggaccaaccaactctggaaatctgttctgcaaacacatgctcacacacacacacacaaatagtataaacaattttaaatttcatttaaaaataatttgtaaacaaaatcattagcacaggttttagaaagagcctcttggtgacatcaagttgatgctgtagatggggtatcattcctgaggacccaaaaccgggtctcagcctttccccattctgagagttctctcttttctcagccactagctgaagagtagagtggctcagcactgggctcttgagttcccaagtcctacaactggtcagcctgactactaaccagccatgaagaaacaaggagtggatgggctgagtctgctgggatgggagtggagttagtaagtggccatggatgtaatgaccccagcaatgctggctagaaggcatgcctcctttccttgtctggagacggaacgggagggatcatcttgtactcacagaagggagaacattctagctggttgggccaaaatgtgcaagttcacctggaggtggtggtgcatgcttttaactccagtactcaggaggcagggccaggtggatctctgtgagttcaagaccagcctgcactatggagagagttttgggacagccagagttacacagaaaaatcctggtggaaaatctgaaagaaagagagaaagaaagaaagaaagaaaggaagaaagaaagaaagagtggcaggcaggcaggcaggaggaaggaaggaaggaaggaaggaaggaaggaaggaaggaaggaaaataggtgcgacttcaagatccggagttacaagcagaatgcactgtttccctaacagggccaagtgttttgagtaactgaaggtgggcatgatgcctgggaagcagaaacaagccaggcagatgcaccccttgccttgcttccgaagggctgcagtagcatggaaaacatggaaaacaaccaatccattccctttgctgatataacaggctccaaagccaaaacctgtcactggaggctcaagagcagatctccagccaagaggcaaaggaatgggggaagctggagggcctccctctggttatccaggcttctgaaggttcaagcaaagaaagggttacaaccttaaaaggagagcgtcccggggtatgggtagaagactgctccaccccgacccccagggtccctaaccgtcttttccctgggcgagtcagcccaatcacaggactgagagtgcctctttagtagcagcaagccacttcggacacccaaatggaacacctccagtcagccctcgccgaccaccccaccccctccatccttttccctcagcctccgattggctgaatctagagtccctccctgctcccccctctctccccacccctggtgaaaactgcgggcttcagcgctgggtgcagcaactggaggcgttggcgcaccaggaggaggctgcagctaggggagtccaggtgagagcaggccgacgggagggacccgcacatgcaaggaccgccgcagggcgaggatgcaagccttccccagctacagttttgggaaaggataccagggcgctcctatatgggggcgcgggaactggggaaagaaggtgctcccaggtcgaggtgggagaggaaggcagtgcggggtcacgggctttctccctgctaacggacgctttcgaagagtgggtgccggaggagaaccatgaggaaggacatcaaggacagcctttggtccccaagctcaaatcgctttagtggtgcgaatagagggaggaggtgggtggcaaactggagggagtccccagcgggtgacctcgtggctggctgggtgcggggcaccgcaggtaagaaaaccgcaatgttgcgggaggggactgggtggcaggcgcgggggaggggaaagctagaaaggatgcgagggagcggaggggggagggagcgggagaatctcaactggtagaggaagattaaaatgaggaaatagcatcagggtggggttagccaagccgggcctcagggaaagggcgcaaagtttgtctgggtgtgggcttaggtgggctgggtatgagattcggggcgccgaaaacactgctgcgcctctgccaaatcacgctacccctgtatctagttctgccaggcttctccagccccagccccaattcttttctctagtgttcccccttccctcccctgaatctcaagcccacactccctcctccataacccactgttatcaaatctaagtcatttgccacccaacaaccatcaggaggcggaagcagacgggaggagtttgagatcaacttgggctacatcacgagttccaggctcaccaaggcttcttaaggagaccttgtctctaaaattaattaattaattaattaatagtcccctttctctgccacagaaccttgggatctggctcctggtcgcagctccccccaccccaggctgacattcactgccatagcccatccggaaatcctagtctatttccccatggatcttgaactgcagagagaatggcagagtggcccgccctgtgcaaaggatgttcctagcctaggtggagctcgcgaactcgcagactgtgcctctcttgggcaaggacaggctagacagcctgccggtgtgttgagctagggcactgtggggaaggcagagaacctgtgcagggcagcaatgaacacaggaccagaaaactgcagccctaggaacactcaagagctggccatttgcaagcatctctggcctccgtgcttctcactcatgtcccatgtcttatacaggcctctgtggcacctcgcttgcctgatctcatccctagccgttaagctttctgcatgacttatcacttggggcataatgctggatacctaccattttcttagaccccatcaaaatcctatttgagtgtacggttcggagaacctcatttatccggtaaatgtcttttactctgctctcagggagctgaggcaggacatcctgagatacattgggagaggagatacagtttcaataaaataataggttgggtggaggtacatgcctataatgccaccactcaggaaatggtggcagcttcgtgagtttgaggccaacccaagaaacatagtgaaaccctgtcagtaaataagtaagcaagtatttgagtatctactatatgctagggctgacctggacattaggggtcatcttctgaacaaactagtgcttgagggaggtatttggggtttttgtttgtttaatggatctgaatgagttccagagactggctacacagcgatatgactgagcttaacacccctaaagcatacagtcagaccaattagacaataaaaggtatgtatagcttaccaaataaaaaaattgtattttcaagagagtgtctgtctgtgtagccctggctgttcttgaactcactctgtagaccaggctggcctggaaatccatctgcctgcctctgcctctctgcctctctgcctctctgcctctctctctgcctctctctgcctctctctgcccctctctgcccctctctgcccctctctgccgccctctgccttttgccctctgccctctgttctctggcctctgccctctgccctctggcctctggcctctgcctctgcctcttgagtgctggaatcaaaggtgtgagctctgtaggtcttaagttccagaagaaagtaatgaagtcacccagcagggaggtgctcagggacagcacagacacacacccaggacataggctcccacttccttggctttctctgagtggcaaaggaccttaggcagtgtcactccctaagagaaggggataaagagaggggctgaggtattcatcatgtgctccgtggatctcaagccctcaaggtaaatggggacccacctgtcctaccagctggctgacctgtagctttccccaccacagaatccaagtcggaactcttggcacctagaggatctcgaggtccttcctctgcagaggtcttgcttctcccggtcagctgactccctccccaagtccttcaaatatctcagaacatggggagaaacggggaccttgtccctcctaaggaaccccagtgctgcatgccatcatcccccccaccctcgcccccacccccgccacttctccctccatgcataccactagctgtcattttgtactctgtatttattccagggctgcttctgattatttagtttgttctttccctggagacctgttagaacataagggcgtatggtgggtaggggaggcaggatatcagtccctggggcgagttcctccctgccaaccaagccagatgcctgaaagagatatggatgagggaagttggactgtgcctgtacctggtacagtcatactctgttgaaagaatcatcggggaggggggggggctcaagaggggagagctctgctgagcctttgtggaccatccaatgaggatgagggcttagattctaccaggtcattctcagccaccacacacaagcgctctgccatcactgaagaagccccctagggctcttgggccagggcacactcagtaaagatgcaggttcagtcagggaatgatggggaaaggggtaggaggtgggggagggatcaccccctcctctaaaacacgagcctgctgtctccaaaggcctctgcctgtagtgagggtggcagaagaagacaaggagccagaactctgactccaggatctaagtccgtgcaggaaggggatcctagaaccatctggttggacccagcttaccaagggagagcctttattcttctttcccttgcccctctgtgccagcccctcttgctgtccctgatcccccagacagcgagagtcttgcaacctgcctcttccaagacctcctaatctcaggggcaggcggtggagtgagatccggcgtgcacactttttggaagatagctttcccaaggatcctctcccccactggcagctctgcctgtcccatcaccatgtataataccaccactgctacagcatctcaccgaggaaagaaaactgcacaataaaaccaagcctctggagtgtgtcctggtgtctgtctcttctgtgtcctggcgtctgtctcttctgtgttcttccaaggtcagaaacaaaaaccacacacttcaacctggatggctcggctgagcacttctgtgtgcagaaggtccaaccagactctggggtaccccggccctccctattcccttgcctcctgtctcccgctttttatagctccctatgctgggcttctctggagagtgaaatctttgcccaaatcaatgcgcattctctctgctgagtcatctggcgacagcagttgagttcacccgccaacacatgggcccagctatgtagccgaaccctggctctggaagtgccagggactttgtgcataagtatgtaccatgcccttttttcacagtcctagctctgcagaagtgcagcctgaaggcctgtctgctgagaggacatgccctggagccctgaaacaggcacagtgggaggaggaacggaggatgacaggcatcaggccctcagtccaaaagcaaccacttgagaatgggctggagtacgaaacatggggtcccgtccctggatccctcctcaaagagtaataagtaaaatataaacaggtaccccaggccgttctgggtttgggttgtaatgggatccatttgcagagaactattgagacagcccagccgtactgtgacaggcaatgtgggggaggaggttgaatcacttggtatttagcatgaatagaataattccctgaacatttttcttaaacatccatatctaaattaccaccactcgctcccagtcttcctgcctttgcgccagcctcctgtctggccatgcctgaagaaggctggagaagccacccacctcaggccatgacactgccagccacttggcaggtgcagccaaacctgagctgtcccagaaagggacattctcaagacccaggcaccctgatcagcactgacttggagctacaagtgtcatgccagaaaagtctctaagaaaaccttttcagggaaaagggggtgactcaacaccgggcaagtttgggaagccccacccttcgagtgatggaagagcagataggaagcctcagaagagagacaccggcacccaggtaacgttcctcatgtggtctctgtcacactaggtgctcttccctggacatctccgtgaccacactctcagttcttagggagatgcgggtgctctctgaggctatctcagagttgcagattctgaggcctagagtgactacagtcagcctaggaagccacagaggactgtggaccaggagggcagaagaggagaagggaagaaaaaccatcagataggacttgcaatgaaactaacccaagacaatcataatgcagacaggaatgttaaaggcgttcagcagc